European Patent Specification EP 3 591 057 B9, published July 19, 2023. Title: INDUCIBLE COEXPRESSION SYSTEM. Applicant: AbSci, LLC. The sequence listing filed with the application follows.

SEQUENCE LISTING (53 sequences)

SEQ ID NO: 1 - DNA, 1526 bp, Mus musculus
ctgactctaaccatggaatggagttggatatttctctttctcctgtcaggaactgcaggtgtccactctgaggtccagctgcagcagtctggacctgagctgataaagcctggggcttcagtgaagatgtcctgcaaggcttctggatacacattcactagctatgttatgcactgggtgaagcagaagcctgggcagggccttgagtggattggatatattaatccttacaatgatggtactaagtacaatgagaagttcaaaggcaaggccacactgacttcagacaaatcctccagcacagcctacatggagctcagcagcctgacctctgaggactctgcggtctattactgtgcaagagggacttattactacggtagtagggtatttgactactggggccaaggcaccactctcacagtctcctcagccaaaacgacacccccatctgtctatccactggcccctggatctgctgcccaaactaactccatggtgaccctgggatgcctggtcaagggctatttccctgagccagtgacagtgacctggaactctggatccctgtccagcggtgtgcacaccttcccagctgtcctgcagtctgacctctacactctgagcagctcagtgactgtcccctccagcacctggcccagcgagaccgtcacctgcaacgttgcccacccggccagcagcaccaaggtggacaagaaaattgtgcccagggattgtggttgtaagccttgcatatgtacagtcccagaagtatcatctgtcttcatcttccccccaaagcccaaggatgtgctcaccattactctgactcctaaggtcacgtgtgttgtggtagacatcagcaaggatgatcccgaggtccagttcagctggtttgtagatgatgtggaggtgcacacagctcagacgcaaccccgggaggagcagttcaacagcactttccgctcagtcagtgaacttcccatcatgcaccaggactggctcaatggcaaggagttcaaatgcagggtcaacagtgcagctttccctgcccccatcgagaaaaccatctccaaaaccaaaggcagaccgaaggctccacaggtgtacaccattccacctcccaaggagcagatggccaaggataaagtcagtctgacctgcatgataacagacttcttccctgaagacattactgtggagtggcagtggaatgggcagccagcggagaactacaagaacactcagcccatcatggacacagatggctcttacttcgtctacagcaagctcaatgtgcagaagagcaactgggaggcaggaaatactttcacctgctctgtgttacatgagggcctgcacaaccaccatactgagaagagcctctcccactctcctggtaaatgatcccagtgtccttggagccctctggtcctacaggactctgacacctacctccacccctccctgtataaataaagcacccagcactgccttgggaccctgcaataaaaaaaaaaaaaaaa

SEQ ID NO: 2 - protein, 464 aa, Mus musculus
MEWSWIFLFLLSGTAGVHSEVQLQQSGPELIKPGASVKMSCKASGYTFTSYVMHWVKQKPGQGLEWIGYINPYNDGTKYNEKFKGKATLTSDKSSSTAYMELSSLTSEDSAVYYCARGTYYYGSRVFDYWGQGTTLTVSSAKTTPPSVYPLAPGSAAQTNSMVTLGCLVKGYFPEPVTVTWNSGSLSSGVHTFPAVLQSDLYTLSSSVTVPSSTWPSETVTCNVAHPASSTKVDKKIVPRDCGCKPCICTVPEVSSVFIFPPKPKDVLTITLTPKVTCVVVDISKDDPEVQFSWFVDDVEVHTAQTQPREEQFNSTFRSVSELPIMHQDWLNGKEFKCRVNSAAFPAPIEKTISKTKGRPKAPQVYTIPPPKEQMAKDKVSLTCMITDFFPEDITVEWQWNGQPAENYKNTQPIMDTDGSYFVYSKLNVQKSNWEAGNTFTCSVLHEGLHNHHTEKSLSHSPGK

SEQ ID NO: 3 - DNA, 958 bp, Mus musculus
ctttttgtatcaagttctcagaatgaggtgcctagctgagttcctggggctgcttgtgctctggatccctggagccattggggatattgtgatgactcaggctgcaccctctatacctgtcactcctggagagtcagtatccatctcctgcaggtctagtaagagtctcctgaatagtaatggcaacacttacttgtattggttcctgcagaggccaggccagtctcctcagctcctgatatatcggatgtccaaccttgcctcaggagtcccagacaggttcagtggcagtgggtcaggaactgctttcacactgagaatcagtagagtggaggctgaggatgtgggtgtttattactgtatgcaacatctagaatatccgttcacgttcggtgctgggaccaagctggagctgaaacgggctgatgctgcaccaactgtatccatcttcccaccatccagtgagcagttaacatctggaggtgcctcagtcgtgtgcttcttgaacaacttctaccccaaagacatcaatgtcaagtggaagattgatggcagtgaacgacaaaatggcgtcctgaacagttggactgatcaggacagcaaagacagcacctacagcatgagcagcaccctcacgttgaccaaggacgagtatgaacgacataacagctatacctgtgaggccactcacaagacatcaacttcacccattgtcaagagcttcaacaggaatgagtgttagagacaaaggtcctgagacgccaccaccagctccccagctccatcctatcttcccttctaaggtcttggaggcttccccacaagcgacctaccactgttgcggtgctccaaacctcctccccacctccttctcctcctcctccctttccttggcttttatcatgctaatatttgcagaaaatattcaataaagtgagtctttgcacttgaaaaaaaa

SEQ ID NO: 4 - protein, 239 aa, Mus musculus
MRCLAEFLGLLVLWIPGAIGDIVMTQAAPSIPVTPGESVSISCRSSKSLLNSNGNTYLYWFLQRPGQSPQLLIYRMSNLASGVPDRFSGSGSGTAFTLRISRVEAEDVGVYYCMQHLEYPFTFGAGTKLELKRADAAPTVSIFPPSSEQLTSGGASVVCFLNNFYPKDINVKWKIDGSERQNGVLNSWTDQDSKDSTYSMSSTLTLTKDEYERHNSYTCEATHKTSTSPIVKSFNRNEC

SEQ ID NO: 5 - DNA, 1429 bp, Artificial Sequence
  Optimized coding sequence for the mouse anti-human CD19 IgG1 heavy chain
ttgggctagcaggaggaattcaccatggaatggtcgtggatttttctgtttctgctgtcgggtacggcgggcgttcatagcgaagttcaactgcaacaaagcggtccggaactgattaaaccgggcgcgagcgtgaagatgtcttgcaaagccagtggttacacctttacgtcttatgtgatgcattgggttaaacagaagccgggccaaggtctggaatggattggctacatcaacccgtacaacgatggtaccaagtacaacgaaaagttcaagggcaaagcaaccctgacgagtgacaaaagctctagtacggcttatatggaactgtcctcactgacctcagaagattcggcagtgtattactgcgctcgtggcacgtattactatggttcccgcgtttttgattactggggccagggtaccacgctgaccgtttcgagcgcgaaaaccacgccgccgagcgtctatccgctggcaccgggttcggcagcacagacgaatagcatggtgaccctgggctgtctggttaaaggttactttccggaaccggtgaccgttacgtggaacagcggctctctgtctagtggtgtccatacgttcccggcggtgctgcagtctgatctgtataccctgtcctcatcggtcacggtgccgagctctacctggccgagtgaaaccgtcacgtgcaacgtggcacacccggcaagttccaccaaagttgataaaaagattgtcccgcgtgactgcggctgtaaaccgtgcatctgtaccgtgccggaagtttcatcggtctttattttcccgccgaagccgaaagatgtcctgaccatcacgctgaccccgaaggtgacctgtgtggttgtcgacatttctaaagatgacccggaagttcagtttagttggttcgtcgatgacgttgaagtccatacggcgcagacccaaccgcgtgaagaacagtttaatagcaccttccgcagtgtgtccgaactgccgatcatgcaccaagactggctgaatggcaaggaatttaaatgccgtgttaactcggcagctttcccggccccgattgaaaagacgatcagcaagaccaaaggtcgcccgaaagcaccgcaggtgtataccattccgccgccgaaagaacaaatggctaaggataaagttagcctgacgtgtatgattaccgatttctttccggaagacatcaccgtggaatggcagtggaacggccaaccggccgaaaactataaaaatacgcagccgatcatggataccgacggttcctactttgtgtattcaaagctgaacgttcaaaaatccaattgggaagccggtaacacgttcacctgttcagttctgcacgaaggtctgcacaatcaccatacggaaaagtcgctgtcccactcgccgggtaaataaaagcttggct

SEQ ID NO: 6 - DNA, 757 bp, Artificial Sequence
  Optimized coding sequence for the mouse anti-human CD19 IgG1 light chain
ttgggctagcaggaggaattcaccatggctcgttgtctggcggaatttctgggtctgctggttctgtggatcccgggcgcgattggcgatattgttatgacgcaagcggctccgtctattccggttaccccgggtgaaagcgtctctatcagttgccgcagctctaaatcgctgctgaacagcaatggtaacacctatctgtactggtttctgcagcgtccgggtcagagcccgcaactgctgatttatcgcatgtctaatctggcaagtggtgtcccggatcgtttttccggttcaggttcgggtacggcattcaccctgcgtatctcccgcgttgaagccgaagacgtcggcgtgtattactgcatgcagcatctggaatacccgtttacgttcggtgcaggcaccaaactggaactgaaacgcgctgatgcagcaccgaccgtgagcattttcccgccgagttccgaacaactgacctccggcggtgcatcagtggtttgttttctgaacaacttctacccgaaagatatcaacgtgaaatggaaaatcgacggttcggaacgtcagaatggcgttctgaacagctggacggatcaagacagtaaagattccacctactcaatgtcatcgaccctgacgctgaccaaagacgaatatgaacgccataactcttacacgtgcgaagctacccacaaaacgagcacctctccgatcgttaaaagttttaatcgtaacgaatgttaaaagcttggct

SEQ ID NO: 7 - DNA, 5874 bp, Artificial Sequence
  pPRO33 vector
atcgattcagcttttcagccgccgccagaacgtcgtccggctgatgcctaaataattcgccgctgctgttttatcgccattaaatttctccagtgcctgttgtggtgtcagtaagcgtggagcgggagttttcgccgactcgcgcgccagttccggcagtagcagttgcataaactgcggcgttaaatccggcgtcggttccacacttaaaaacagcgccagtcgttccatcatattgcgcagttcacgaatattgcctggccagtcgtagtgcagcagcacagtttcacttgcctgtaacccctggcgtaatgcagcagaaaatggggcggagagcgccgccagagacactttcaaaaagctttccgccagcggaagaatatccgccacccgctcgcgcagtggtggcaattgcagacgcaaaatactcagccgataaaacagatcacggcgaaaacgtccttgctgcatatcttcttccagattgcagtgagtggcgctaatgacccgtacatctaccggaacaggctgatgcccgccgacgcgggtgacctctttttcttccagcacccgcagcagccgggtctgcaaaggtagcggcatttcgccaatctcatccagaaacagcgtaccgccgtgggcaatttcgaacagcccggcgcgacctccgcgtcgcgagccggtaaacgccccttcctcatagccaaacagttctgcttccagcagcgattcggcaatcgccccgcagttgacggcaacaaacggatgcgactttttgccctgtcgcgcatcgtggcgggcaaaatattcccgatgaatcgcctgggccgccagctctttgcccgtccccgtttccccctcaatcaacaccgccgcactggagcgggcatacagcaaaatagtctgccgtacttgttccatctgtggtgattgaccgagcatatcgcccagcacgtaacgagtacgcagggcgttgcgggtggcatcgtgagtgttatggcgtaacgacatgcgcgtcatatccagcgcatcgctgaacgcctggcgcacggtggcggcggaatagataaaaattccggtcattccggcttcttctgccaaatcggtaatcagccctgcgccgaccaccgcttcggtgccgttagcttttagctcgttaatctgcccgcgtgcgtcttcctcggtaatgtagctacgttggtcgaggcgcaaattaaaggttttttgaaacgccaccagcgctggaatggtttcctgataggtgacaacgccgatagaagaggtgagttttccggcttttgccagtgcctgtaacacatcgtagccgctcggtttaatcaaaataactggcactgacaggcggcttttcaggtacgcgccgttagagccagccgcgatgatggcgtcacagcgttcgtttgccagtttcttgcggatgtaggtcactgctttttcaaagccaagctgaataggggtaatgttcgccaggtgatcaaactcgaggctgatatcgcgaaacagctcgaacaggcgcgttacagataccgtccagataaccggtttgtcgtcattaagccgtggtggatgtgccatagcgcaccgcaaagttaagaaaccgaatattgggtttagtcttgtttcataattgttgcaatgaaacgcggtgaaacattgcctgaaacgttaactgaaacgcatatttgcggattagttcatgactttatctctaacaaattgaaattaaacatttaattttattaaggcaattgtggcacaccccttgctttgtctttatcaacgcaaataacaagttgataacaagctagcgaattcgagctcggtacccggggatcctctagagtcgacctgcaggcatgcaagcttggctgttttggcggatgagagaagattttcagcctgatacagattaaatcagaacgcagaagcggtctgataaaacagaatttgcctggcggcagtagcgcggtggtcccacctgaccccatgccgaactcagaagtgaaacgccgtagcgccgatggtagtgtggggtctccccatgcgagagtagggaactgccaggcatcaaataaaacgaaaggctcagtcgaaagactgggcctttcgttttatctgttgtttgtcggtgaacgctctcctgagtaggacaaatccgccgggagcggatttgaacgttgcgaagcaacggcccggagggtggcgggcaggacgcccgccataaactgccaggcatcaaattaagcagaaggccatcctgacggatggcctttttgcgtttctacaaactcttttgtttatttttctaaatacattcaaatatgtatccgctcatgagacaataaccctgataaatgcttcaataatattgaaaaaggaagagtatgagtattcaacatttccgtgtcgcccttattcccttttttgcggcattttgccttcctgtttttgctcacccagaaacgctggtgaaagtaaaagatgctgaagatcagttggggcaaactattaactggcgaactacttactctagcttcccggcaacaattaatagactggatggaggcggataaagttgcaggaccacttctgcgctcggcccttccggctggctggtttattgctgataaatctggagccggtgagcgtgggtctcgcggtatcattgcagcactggggccagatggtaagccctcccgtatcgtagttatctacacgacggggagtcaggcaactatggatgaacgaaatagacagatcgctgagataggtgcctcactgattaagcattggtaactgtcagaccaagtttactcatatatactttagattgatttacgcgccctgtagcggcgcattaagcgcggcgggtgtggtggttacgcgcagcgtgaccgctacacttgccagcgccctagcgcccgctcctttcgctttcttcccttcctttctcgccacgttcgccggctttccccgtcaagctctaaatcgggggctccctttagggttccgatttagtgctttacggcacctcgaccccaaaaaacttgatttgggtgatggttcacgtagtgggccatcgccctgatagacggtttttcgccctttgacgttggagtccacgttctttaatagtggactcttgttccaaacttgaacaacactcaaccctatctcgggctattcttttgatttataagggattttgccgatttcggcctattggttaaaaaatgagctgatttaacaaaaatttaacgcgaattttaacaaaatattaacgtttacaatttaaaaggatctaggtgaagatcctttttgataatctcatgaccaaaatcccttaacgtgagttttcgttccactgagcgtcagaccccgtagaaaagatcaaaggatcttcttgagatcctttttttctgcgcgtaatctgctgcttgcaaacaaaaaaaccaccgctaccagcggtggtttgtttgccggatcaagagctaccaactctttttccgaaggtaactggcttcagcagagcgcagataccaaatactgtccttctagtgtagccgtagttaggccaccacttcaagaactctgtagcaccgcctacatacctcgctctgctaatcctgttaccagtcaggcatttgagaagcacacggtcacactgcttccggtagtcaataaaccggtaaaccagcaatagacataagcggctatttaacgaccctgccctgaaccgacgaccgggtcgaatttgctttcgaatttctgccattcatccgcttattatcacttattcaggcgtagcaccaggcgtttaagggcaccaataactgccttaaaaaaattacgccccgccctgccactcatcgcagtactgttgtaattcattaagcattctgccgacatggaagccatcacagacggcatgatgaacctgaatcgccagcggcatcagcaccttgtcgccttgcgtataatatttgcccatggtgaaaacgggggcgaagaagttgtccatattggccacgtttaaatcaaaactggtgaaactcacccagggattggctgagacgaaaaacatattctcaataaaccctttagggaaataggccaggttttcaccgtaacacgccacatcttgcgaatatatgtgtagaaactgccggaaatcgtcgtggtattcactccagagcgatgaaaacgtttcagtttgctcatggaaaacggtgtaacaagggtgaacactatcccatatcaccagctcaccgtctttcattgccatacggaattccggatgagcattcatcaggcgggcaagaatgtgaataaaggccggataaaacttgtgcttatttttctttacggtctttaaaaaggccgtaatatccagctgaacggtctggttataggtacattgagcaactgactgaaatgcctcaaaatgttctttacgatgccattgggatatatcaacggtggtatatccagtgatttttttctccattttagcttccttagctcctgaaaatctcgataactcaaaaaatacgcccggtagtgatcttatttcattatggtgaaagttggaacctcttacgtgccgatcaacgtctcattttcgccaaaagttggcccagggcttcccggtatcaacagggacaccaggatttatttattctgcgaagtgatcttccgtcacaggtatttattcggcgcaaagtgcgtcgggtgatgctgccaacttactgatttagtgtatgatggtgtttttgaggtgctccagtggcttctgtttctatcagctgtccctcctgttcagctactgacggggtggtgcgtaacggcaaaagcaccgccggacatcagcgctagcggagtgtatactggcttactatgttggcactgatgagggtgtcagtgaagtgcttcatgtggcaggagaaaaaaggctgcaccggtgcgtcagcagaatatgtgatacaggatatattccgcttcctcgctcactgactcgctacgctcggtcgttcgactgcggcgagcggaaatggcttacgaacggggcggagatttcctggaagatgccaggaagatacttaacagggaagtgagagggccgcggcaaagccgtttttccataggctccgcccccctgacaagcatcacgaaatctgacgctcaaatcagtggtggcgaaacccgacaggactataaagataccaggcgtttccccctggcggctccctcgtgcgctctcctgttcctgcctttcggtttaccggtgtcattccgctgttatggccgcgtttgtctcattccacgcctgacactcagttccgggtaggcagttcgctccaagctggactgtatgcacgaaccccccgttcagtccgaccgctgcgccttatccggtaactatcgtcttgagtccaacccggaaagacatgcaaaagcaccactggcagcagccactggtaattgatttagaggagttagtcttgaagtcatgcgccggttaaggctaaactgaaaggacaagttttggtgactgcgctcctccaagccagttacctcggttcaaagagttggtagctcagagaaccttcgaaaaaccgccctgcaaggcggttttttcgttttcagagcaagagattacgcgcagaccaaaacgatctcaagaagatcatcttattaatcagataaaatatttgctcatgagcccgaagtggcgagcccgatcttccccatcggtgatgtcggcgatataggcgccagcaaccgcacctgtggcgccggtgatgccggccacgatgcgtccggcgtagaggatctgctcatgtttgacagcttatc

SEQ ID NO: 8 - DNA, 36 bp, Artificial Sequence
  IgG1HC Fc forward primer
ttcaccatggaagtttcatcggtctttattttcccg

SEQ ID NO: 9 - DNA, 32 bp, Artificial Sequence
  IgG1HC Fc reverse primer
agccaagcttttatttacccggcgagtgggac

SEQ ID NO: 10 - DNA, 19 bp, Artificial Sequence
  pBAD24/33 forward primer
ctgtttctccatacccgtt

SEQ ID NO: 11 - DNA, 17 bp, Artificial Sequence
  pBAD24/33 reverse primer #1
ctcatccgccaaaacag

SEQ ID NO: 12 - DNA, 17 bp, Artificial Sequence
  pBAD24/33 reverse primer #2
ggctgaaaatcttctct

SEQ ID NO: 13 - protein, 370 aa, Artificial Sequence
  P. chrysosporium MnP-H4 amino acid sequence, without signal peptide
MAITRAAPTAESAVCPDGTRVTNAACCAFIPLAQDLQETLFQGDCGEDAHEVIRLTFHDAIAISQSLGPQAGGGADGSMLHFPTIEPNFSANSGIDDSVNNLLPFMQKHDTISAADLVQFAGAVALSNCPGAPRLEFMAGRPNTTIPAVEGLIPEPQDSVTKILQRFEDAGNFSPFEVVSLLASHTVARADKVDETIDAAPFDSTPFTFDTQVFLEVLLKGTGFPGSNNNTGEVMSPLPLGSGSDTGEMRLQSDFALARDERTACFWQSFVNEQEFMAASFKAAMAKLAILGHSRSSLIDCSDVVPVPKPAVNKPATFPATKGPKDLDTLTCKALKFPTLTSDPGATETLIPHCSNGGMSCPGVQFDGPA

SEQ ID NO: 14 - DNA, 1113 bp, Artificial Sequence
  Optimized coding sequence for P. chrysosporium MnP-H4, without signal peptide
atggcaatcacgagagcagcaccaaccgcagaatccgcagtatgtccagacggtaccagagtgacgaatgcagcgtgttgcgcgttcattccgctggcgcaggatctgcaggaaaccctgttccaaggcgattgcggcgaggacgcgcacgaggtcattcgcctgacctttcacgatgccattgcaatcagccagtctttgggtccgcaagcgggtggtggcgcggacggcagcatgttgcactttccgaccatcgagccgaatttctcggccaatagcggtattgacgatagcgttaacaacctgttgccgtttatgcaaaagcatgacaccatcagcgctgcggacctggttcagttcgcaggcgccgtggcgctgagcaactgtcctggtgcgccacgtctggagttcatggcgggtcgcccgaataccacgatcccggcagttgaaggtctgattccggagccgcaggacagcgtcaccaaaattctgcagcgtttcgaggatgccggtaactttagcccgttcgaggtcgtgagcctgttggcgagccatacggtggcgcgtgctgacaaagttgatgaaaccatcgacgccgctccgttcgacagcaccccgtttacgtttgatacccaggttttcctggaagttctgttgaaaggcaccggctttccgggttccaataacaacaccggtgaagtcatgtctccgctgcctctgggctcgggtagcgatactggtgagatgcgcctgcaaagcgactttgctctggcccgtgatgagcgtaccgcgtgcttctggcagtccttcgtcaacgaacaagagtttatggcggccagctttaaggctgcgatggcaaaactggcaattctgggccatagccgttccagcctgatcgattgcagcgacgtggttccggtgccgaagcctgcggtcaataagccggcgaccttcccggcgaccaaaggcccgaaggacctggatactctgacgtgtaaagcgctgaagtttccgacgctgacgtctgatccgggtgccacggagactctgatcccgcactgcagcaatggtggcatgagctgcccgggtgtgcaattcgacggtccggcgtaa

SEQ ID NO: 15 - protein, 370 aa, Artificial Sequence
  P. chrysosporium MnP-H4 A60C/A75C amino acid sequence, without signal peptide
MAITRAAPTAESAVCPDGTRVTNAACCAFIPLAQDLQETLFQGDCGEDAHEVIRLTFHDCIAISQSLGPQAGGGCDGSMLHFPTIEPNFSANSGIDDSVNNLLPFMQKHDTISAADLVQFAGAVALSNCPGAPRLEFMAGRPNTTIPAVEGLIPEPQDSVTKILQRFEDAGNFSPFEVVSLLASHTVARADKVDETIDAAPFDSTPFTFDTQVFLEVLLKGTGFPGSNNNTGEVMSPLPLGSGSDTGEMRLQSDFALARDERTACFWQSFVNEQEFMAASFKAAMAKLAILGHSRSSLIDCSDVVPVPKPAVNKPATFPATKGPKDLDTLTCKALKFPTLTSDPGATETLIPHCSNGGMSCPGVQFDGPA

SEQ ID NO: 16 - DNA, 1113 bp, Artificial Sequence
  Optimized coding sequence for P. chrysosporium MnP-H4 A60C/A75C, without signal peptide
atggcaatcacgagagcagcaccaaccgcagaatccgcagtatgtccagacggtaccagagtgacgaatgcagcgtgttgcgcgttcattccgctggcgcaggatctgcaggaaaccctgttccaaggcgattgcggcgaggacgcgcacgaggtcattcgcctgacctttcacgattgcattgcaatcagccagtctttgggtccgcaagcgggtggtggctgcgacggcagcatgttgcactttccgaccatcgagccgaatttctcggccaatagcggtattgacgatagcgttaacaacctgttgccgtttatgcaaaagcatgacaccatcagcgctgcggacctggttcagttcgcaggcgccgtggcgctgagcaactgtcctggtgcgccacgtctggagttcatggcgggtcgcccgaataccacgatcccggcagttgaaggtctgattccggagccgcaggacagcgtcaccaaaattctgcagcgtttcgaggatgccggtaactttagcccgttcgaggtcgtgagcctgttggcgagccatacggtggcgcgtgctgacaaagttgatgaaaccatcgacgccgctccgttcgacagcaccccgtttacgtttgatacccaggttttcctggaagttctgttgaaaggcaccggctttccgggttccaataacaacaccggtgaagtcatgtctccgctgcctctgggctcgggtagcgatactggtgagatgcgcctgcaaagcgactttgctctggcccgtgatgagcgtaccgcgtgcttctggcagtccttcgtcaacgaacaagagtttatggcggccagctttaaggctgcgatggcaaaactggcaattctgggccatagccgttccagcctgatcgattgcagcgacgtggttccggtgccgaagcctgcggtcaataagccggcgaccttcccggcgaccaaaggcccgaaggacctggatactctgacgtgtaaagcgctgaagtttccgacgctgacgtctgatccgggtgccacggagactctgatcccgcactgcagcaatggtggcatgagctgcccgggtgtgcaattcgacggtccggcgtaa

SEQ ID NO: 17 - protein, 660 aa, E. coli O157:H7
MSRPQFTSLRLSLLALAVSATLPTFAFATETMTVTATGNARSSFEAPMMVSVIDTSAPENQTATSATDLLRHVPGITLDGTGRTNGQDVNMRGYDHRGVLVLVDGVRQGTDTGHLNGTFLDPALIKRVEIVRGPSALLYGSGALGGVISYDTVDAKDLLQEGQSSGFRVFGTGGTGDHSLGLGASAFGRTENLDGIVAWSSRDRGDLRQSNGETAPNDESINNMLAKGTWQIDSAQSLSGLVRYYNNDAREPKNPQTVEASESSNPMVDRSTIQRDAQLSYKLAPQGNDWLNADAKIYWSEVRINAQNTGSSGEYREQITKGARLENRSTLFADSFASHLLTYGGEYYRQEQHPGGATTGFPQAKIDFSSGWLQDEITLRDLPITLLGGTRYDSYRGSSDGYKDVDADKWSSRAGMTINPTNWLMLFGSYAQAFRAPTMGEMYNDSKHFSIGRFYTNYWVPNPNLRPETNETQEYGFGLRFDDLMLSNDALEFKASYFDTKAKDYISTTVDFAAATTMSYNVPNAKIWGWDVMTKYTTDLFSLDVAYNRTRGKDTDTGEYISSINPDTVTSTLNIPIAHSGFSVGWVGTFADRSTHISSSYSKQPGYGVNDFYVSYQGQQALKGMTTTLVLGNAFDKEYWSPQGIPQDGRNGKIFVSYQW

SEQ ID NO: 18 - DNA, 1276 bp, Artificial Sequence
  MnP-H4 expression construct
gctagcaggaggaattcaccatggcaatcacgagagcagcaccaaccgcagaatccgcagtatgtccagacggtaccagagtgacgaatgcagcgtgttgcgcgttcattccgctggcgcaggatctgcaggaaaccctgttccaaggcgattgcggcgaggacgcgcacgaggtcattcgcctgacctttcacgatgccattgcaatcagccagtctttgggtccgcaagcgggtggtggcgcggacggcagcatgttgcactttccgaccatcgagccgaatttctcggccaatagcggtattgacgatagcgttaacaacctgttgccgtttatgcaaaagcatgacaccatcagcgctgcggacctggttcagttcgcaggcgccgtggcgctgagcaactgtcctggtgcgccacgtctggagttcatggcgggtcgcccgaataccacgatcccggcagttgaaggtctgattccggagccgcaggacagcgtcaccaaaattctgcagcgtttcgaggatgccggtaactttagcccgttcgaggtcgtgagcctgttggcgagccatacggtggcgcgtgctgacaaagttgatgaaaccatcgacgccgctccgttcgacagcaccccgtttacgtttgatacccaggttttcctggaagttctgttgaaaggcaccggctttccgggttccaataacaacaccggtgaagtcatgtctccgctgcctctgggctcgggtagcgatactggtgagatgcgcctgcaaagcgactttgctctggcccgtgatgagcgtaccgcgtgcttctggcagtccttcgtcaacgaacaagagtttatggcggccagctttaaggctgcgatggcaaaactggcaattctgggccatagccgttccagcctgatcgattgcagcgacgtggttccggtgccgaagcctgcggtcaataagccggcgaccttcccggcgaccaaaggcccgaaggacctggatactctgacgtgtaaagcgctgaagtttccgacgctgacgtctgatccgggtgccacggagactctgatcccgcactgcagcaatggtggcatgagctgcccgggtgtgcaattcgacggtccggcgtaatactagagccaggcatcaaataaaacgaaaggctcagtcgaaagactgggcctttcgttttatctgttgtttgtcggtgaacgctctctactagagtcacactggctcaccttcgggtgggcctttctgcgtttatatctaga

SEQ ID NO: 19 - DNA, 2056 bp, Artificial Sequence
  ChuA expression construct
tctagattgacagctagctcagtcctaggtattgtgctagctactagagaaagaggagaaatactagatgtcccgccctcaattcacctcgctccgtttgtctttgctcgcactcgccgtatccgcaacgctgccgacctttgccttcgctaccgaaaccatgaccgttaccgcgaccggcaacgcacgcagctcgttcgaggcgccgatgatggtgagcgtgatcgatacctctgctccggagaaccagacggcgacgagcgctaccgatctgctgcgccacgtgccgggtattacgctggacggtaccggtcgcacgaacggtcaagacgtgaacatgcgcggctacgaccatcgcggtgtgctggtcctggtcgatggtgtgcgtcagggtacggataccggtcacttgaatggtacctttctggatccggcgctgattaagcgtgtcgaaatcgtgcgtggcccgtcggcactgctgtatggtagcggtgcgctgggcggtgtgatcagctacgataccgtcgatgcgaaagacctgttgcaagagggtcaaagctccggtttccgcgtttttggtactggtggtaccggtgaccatagcctgggcctgggcgcgagcgcgtttggtcgcacggaaaacctggatggcatcgttgcgtggagcagccgtgatcgtggtgacttgcgccagtctaatggcgaaacggcccctaacgatgaaagcattaacaacatgctggccaagggtacgtggcagatcgatagcgcgcagagcctgagcggcctggtccgttactacaacaacgacgcgcgtgagccgaaaaacccgcagacggtcgaggcgagcgagagcagcaacccgatggtggaccgtagcaccattcaacgtgatgcccaactgagctataagctggcaccgcaaggtaatgactggctgaatgcggatgcgaaaatctactggagcgaagttcgcatcaatgcacagaatacgggtagctctggcgagtaccgtgaacagattaccaaaggtgcacgtctggagaatcgttctacgctgtttgctgacagcttcgcttcgcatctgctgacgtatggtggcgagtattatcgtcaggaacaacacccaggtggtgcgaccacgggtttcccgcaggcgaagatcgattttagcagcggctggctgcaagatgagatcaccttgcgtgacttgccgattaccctgctgggtggtacgcgttatgacagctaccgtggcagcagcgacggttacaaagacgtcgatgcagataaatggagctcccgtgccggcatgaccattaatccgaccaattggctgatgctgttcggcagctatgcgcaagcgttccgtgccccaaccatgggtgagatgtacaatgacagcaagcatttcagcattggtcgcttctacacgaattactgggtgccgaacccgaatctgcgtccggagactaatgaaacccaggagtatggttttggcctgcgctttgatgatctgatgctgagcaacgacgccctggaattcaaggcgagctactttgacactaaagccaaagactacattagcactacggttgattttgcggctgctaccaccatgtcctataatgttccaaacgcaaagatttggggctgggacgtcatgaccaagtacaccaccgacctgtttagcttggatgttgcatacaatcgcacccgtggcaaagacaccgataccggcgaatacatcagcagcatcaatccggacaccgttacgtccaccctgaacatcccgattgcgcacagcggtttcagcgttggttgggttggtacgtttgcggatcgctccacccacatctcgtcgtcttatagcaagcaaccgggctacggcgtgaatgatttctatgtgagctatcagggccagcaagccctgaaaggtatgacgactaccctggttctgggcaacgcattcgacaaagagtattggagcccgcagggcattccgcaggacggtcgtaacggcaagattttcgtttcctaccaatggtaagtcgac

SEQ ID NO: 20 - DNA, 3326 bp, Artificial Sequence
  MnP-H4 ChuA expression construct
gctagcaggaggaattcaccatggcaatcacgagagcagcaccaaccgcagaatccgcagtatgtccagacggtaccagagtgacgaatgcagcgtgttgcgcgttcattccgctggcgcaggatctgcaggaaaccctgttccaaggcgattgcggcgaggacgcgcacgaggtcattcgcctgacctttcacgatgccattgcaatcagccagtctttgggtccgcaagcgggtggtggcgcggacggcagcatgttgcactttccgaccatcgagccgaatttctcggccaatagcggtattgacgatagcgttaacaacctgttgccgtttatgcaaaagcatgacaccatcagcgctgcggacctggttcagttcgcaggcgccgtggcgctgagcaactgtcctggtgcgccacgtctggagttcatggcgggtcgcccgaataccacgatcccggcagttgaaggtctgattccggagccgcaggacagcgtcaccaaaattctgcagcgtttcgaggatgccggtaactttagcccgttcgaggtcgtgagcctgttggcgagccatacggtggcgcgtgctgacaaagttgatgaaaccatcgacgccgctccgttcgacagcaccccgtttacgtttgatacccaggttttcctggaagttctgttgaaaggcaccggctttccgggttccaataacaacaccggtgaagtcatgtctccgctgcctctgggctcgggtagcgatactggtgagatgcgcctgcaaagcgactttgctctggcccgtgatgagcgtaccgcgtgcttctggcagtccttcgtcaacgaacaagagtttatggcggccagctttaaggctgcgatggcaaaactggcaattctgggccatagccgttccagcctgatcgattgcagcgacgtggttccggtgccgaagcctgcggtcaataagccggcgaccttcccggcgaccaaaggcccgaaggacctggatactctgacgtgtaaagcgctgaagtttccgacgctgacgtctgatccgggtgccacggagactctgatcccgcactgcagcaatggtggcatgagctgcccgggtgtgcaattcgacggtccggcgtaatactagagccaggcatcaaataaaacgaaaggctcagtcgaaagactgggcctttcgttttatctgttgtttgtcggtgaacgctctctactagagtcacactggctcaccttcgggtgggcctttctgcgtttatatctagattgacagctagctcagtcctaggtattgtgctagctactagagaaagaggagaaatactagatgtcccgccctcaattcacctcgctccgtttgtctttgctcgcactcgccgtatccgcaacgctgccgacctttgccttcgctaccgaaaccatgaccgttaccgcgaccggcaacgcacgcagctcgttcgaggcgccgatgatggtgagcgtgatcgatacctctgctccggagaaccagacggcgacgagcgctaccgatctgctgcgccacgtgccgggtattacgctggacggtaccggtcgcacgaacggtcaagacgtgaacatgcgcggctacgaccatcgcggtgtgctggtcctggtcgatggtgtgcgtcagggtacggataccggtcacttgaatggtacctttctggatccggcgctgattaagcgtgtcgaaatcgtgcgtggcccgtcggcactgctgtatggtagcggtgcgctgggcggtgtgatcagctacgataccgtcgatgcgaaagacctgttgcaagagggtcaaagctccggtttccgcgtttttggtactggtggtaccggtgaccatagcctgggcctgggcgcgagcgcgtttggtcgcacggaaaacctggatggcatcgttgcgtggagcagccgtgatcgtggtgacttgcgccagtctaatggcgaaacggcccctaacgatgaaagcattaacaacatgctggccaagggtacgtggcagatcgatagcgcgcagagcctgagcggcctggtccgttactacaacaacgacgcgcgtgagccgaaaaacccgcagacggtcgaggcgagcgagagcagcaacccgatggtggaccgtagcaccattcaacgtgatgcccaactgagctataagctggcaccgcaaggtaatgactggctgaatgcggatgcgaaaatctactggagcgaagttcgcatcaatgcacagaatacgggtagctctggcgagtaccgtgaacagattaccaaaggtgcacgtctggagaatcgttctacgctgtttgctgacagcttcgcttcgcatctgctgacgtatggtggcgagtattatcgtcaggaacaacacccaggtggtgcgaccacgggtttcccgcaggcgaagatcgattttagcagcggctggctgcaagatgagatcaccttgcgtgacttgccgattaccctgctgggtggtacgcgttatgacagctaccgtggcagcagcgacggttacaaagacgtcgatgcagataaatggagctcccgtgccggcatgaccattaatccgaccaattggctgatgctgttcggcagctatgcgcaagcgttccgtgccccaaccatgggtgagatgtacaatgacagcaagcatttcagcattggtcgcttctacacgaattactgggtgccgaacccgaatctgcgtccggagactaatgaaacccaggagtatggttttggcctgcgctttgatgatctgatgctgagcaacgacgccctggaattcaaggcgagctactttgacactaaagccaaagactacattagcactacggttgattttgcggctgctaccaccatgtcctataatgttccaaacgcaaagatttggggctgggacgtcatgaccaagtacaccaccgacctgtttagcttggatgttgcatacaatcgcacccgtggcaaagacaccgataccggcgaatacatcagcagcatcaatccggacaccgttacgtccaccctgaacatcccgattgcgcacagcggtttcagcgttggttgggttggtacgtttgcggatcgctccacccacatctcgtcgtcttatagcaagcaaccgggctacggcgtgaatgatttctatgtgagctatcagggccagcaagccctgaaaggtatgacgactaccctggttctgggcaacgcattcgacaaagagtattggagcccgcagggcattccgcaggacggtcgtaacggcaagattttcgtttcctaccaatggtaagtcgac

SEQ ID NO: 21 - protein, 486 aa, Artificial Sequence
  Humicola insolens PDI amino acid sequence, without signal peptide
MSDVVQLKKDTFDDFIKTNDLVLAEFFAPWCGHCKALAPEYEEAATTLKEKNIKLAKVDCTEETDLCQQHGVEGYPTLKVFRGLDNVSPYKGQRKAAAITSYMIKQSLPAVSEVTKDNLEEFKKADKAVLVAYVDASDKASSEVFTQVAEKLRDNYPFGSSSDAALAEAEGVKAPAIVLYKDFDEGKAVFSEKFEVEAIEKFAKTGATPLIGEIGPETYSDYMSAGIPLAYIFAETAEERKELSDKLKPIAEAQRGVINFGTIDAKAFGAHAGNLNLKTDKFPAFAIQEVAKNQKFPFDQEKEITFEAIKAFVDDFVAGKIEPSIKSEPIPEKQEGPVTVVVAKNYNEIVLDDTKDVLIEFYAPWCGHCKALAPKYEELGALYAKSEFKDRVVIAKVDATANDVPDEIQGFPTIKLYPAGAKGQPVTYSGSRTVEDLIKFIAENGKYKAAISEDAEETSSATETTTETATKSEEAAKETATEHDEL

SEQ ID NO: 22 - DNA, 1487 bp, Artificial Sequence
  PDI expression construct
gctagcaggaggaattcaccatgtctgatgttgtacaactgaagaaagatacgttcgatgactttatcaaaactaatgacttggtgctggcagagtttttcgccccgtggtgtggccactgcaaagctctggctccggagtacgaagaggccgcgaccaccctgaaagaaaagaacatcaaactggcgaaagtggactgtacggaagaaaccgacctgtgtcagcagcacggcgtggaaggttacccgaccctgaaggtgtttcgtggcctggacaatgttagcccgtacaaaggtcaacgtaaggccgcagcgatcaccagctacatgatcaagcagtcgctgcctgcagtctctgaggtgaccaaagataatctggaagagttcaaaaaggcagataaggcggtgctggttgcctatgttgatgcaagcgacaaggcgagcagcgaggtctttacccaggtcgcggagaaattgcgcgataactacccgttcggcagcagctccgatgcagctttggccgaggcggaaggtgtcaaggctccggcgatcgttctgtacaaagatttcgacgagggtaaagcggtgttcagcgaaaagtttgaggtggaagcaattgaaaagttcgcaaaaaccggtgccacgcctttgattggcgaaatcggtccggaaacctattctgactatatgagcgccggtatcccgctggcctacattttcgcagaaacggcagaagagcgcaaagaactgagcgacaagttgaagccaattgcagaggcacagcgtggcgtcatcaactttggtaccattgacgcgaaagcatttggtgcgcatgccggtaacctgaatctgaaaacggacaaatttccggcgtttgcgattcaagaggtggcgaagaaccaaaagtttccgttcgatcaagaaaaagagattaccttcgaggcgatcaaagcgttcgttgacgactttgttgccggtaaaatcgagccgagcattaagagcgagccgatcccggagaagcaggaaggcccggtgaccgtcgtcgtcgcgaagaattacaacgagattgttctggatgacacgaaagacgtcctgattgagttctatgcgccgtggtgcggtcattgcaaagcgctggccccgaaatatgaagagctgggtgcgctgtacgcgaagagcgagtttaaggaccgtgtggttatcgcgaaagtagatgcgaccgccaatgacgttcctgacgagatccaaggcttcccgaccattaaactgtatccggctggtgctaaaggccagccagttacctatagcggtagccgcacggttgaggatctgattaagttcattgccgagaacggcaagtacaaggcggcaatcagcgaggatgcagaagaaacgagctccgcaaccgaaaccacgacggaaaccgctactaagtccgaagaggcggcgaaagaaaccgcgacggagcacgatgagctgtaagtcgac

SEQ ID NO: 23 - protein, 359 aa, Artificial Sequence
  P. chrysosporium MnP-H4 amino acid sequence, mature and "fully truncated"
MAVCPDGTRVTNAACCAFIPLAQDLQETLFQGDCGEDAHEVIRLTFHDAIAISQSLGPQAGGGADGSMLHFPTIEPNFSANSGIDDSVNNLLPFMQKHDTISAADLVQFAGAVALSNCPGAPRLEFMAGRPNTTIPAVEGLIPEPQDSVTKILQRFEDAGNFSPFEVVSLLASHTVARADKVDETIDAAPFDSTPFTFDTQVFLEVLLKGTGFPGSNNNTGEVMSPLPLGSGSDTGEMRLQSDFALARDERTACFWQSFVNEQEFMAASFKAAMAKLAILGHSRSSLIDCSDVVPVPKPAVNKPATFPATKGPKDLDTLTCKALKFPTLTSDPGATETLIPHCSNGGMSCPGVQFDGPA

SEQ ID NO: 24 - DNA, 25 bp, Artificial Sequence
  MnP-H4_FT NcoI forward primer
cgatgaccatggcagtatgtccaga

SEQ ID NO: 25 - DNA, 27 bp, Artificial Sequence
  MnP-H4_FT SalI reverse primer
ccgtctgtcgactataaacgcagaaag

SEQ ID NO: 26 - DNA, 24 bp, Artificial Sequence
  ChuA SalI forward primer
tgcagagtcgacttgacagctagc

SEQ ID NO: 27 - DNA, 31 bp, Artificial Sequence
  ChuA HindIII reverse primer
cgtctaaagcttttaccattggtaggaaacg

SEQ ID NO: 28 - DNA, 7768 bp, Artificial Sequence
  pBAD24-MnP_FT-ChuA expression construct
atcgatgcataatgtgcctgtcaaatggacgaagcagggattctgcaaaccctatgctactccgtcaagccgtcaattgtctgattcgttaccaattatgacaacttgacggctacatcattcactttttcttcacaaccggcacggaactcgctcgggctggccccggtgcattttttaaatacccgcgagaaatagagttgatcgtcaaaaccaacattgcgaccgacggtggcgataggcatccgggtggtgctcaaaagcagcttcgcctggctgatacgttggtcctcgcgccagcttaagacgctaatccctaactgctggcggaaaagatgtgacagacgcgacggcgacaagcaaacatgctgtgcgacgctggcgatatcaaaattgctgtctgccaggtgatcgctgatgtactgacaagcctcgcgtacccgattatccatcggtggatggagcgactcgttaatcgcttccatgcgccgcagtaacaattgctcaagcagatttatcgccagcagctccgaatagcgcccttccccttgcccggcgttaatgatttgcccaaacaggtcgctgaaatgcggctggtgcgcttcatccgggcgaaagaaccccgtattggcaaatattgacggccagttaagccattcatgccagtaggcgcgcggacgaaagtaaacccactggtgataccattcgcgagcctccggatgacgaccgtagtgatgaatctctcctggcgggaacagcaaaatatcacccggtcggcaaacaaattctcgtccctgatttttcaccaccccctgaccgcgaatggtgagattgagaatataacctttcattcccagcggtcggtcgataaaaaaatcgagataaccgttggcctcaatcggcgttaaacccgccaccagatgggcattaaacgagtatcccggcagcaggggatcattttgcgcttcagccatacttttcatactcccgccattcagagaagaaaccaattgtccatattgcatcagacattgccgtcactgcgtcttttactggctcttctcgctaaccaaaccggtaaccccgcttattaaaagcattctgtaacaaagcgggaccaaagccatgacaaaaacgcgtaacaaaagtgtctataatcacggcagaaaagtccacattgattatttgcacggcgtcacactttgctatgccatagcatttttatccataagattagcggatcctacctgacgctttttatcgcaactctctactgtttctccatacccgtttttttgggctagcaggaggaattcaccatggcagtatgtccagacggtaccagagtgacgaatgcagcgtgttgcgcgttcattccgctggcgcaggatctgcaggaaaccctgttccaaggcgattgcggcgaggacgcgcacgaggtcattcgcctgacctttcacgatgccattgcaatcagccagtctttgggtccgcaagcgggtggtggcgcggacggcagcatgttgcactttccgaccatcgagccgaatttctcggccaatagcggtattgacgatagcgttaacaacctgttgccgtttatgcaaaagcatgacaccatcagcgctgcggacctggttcagttcgcaggcgccgtggcgctgagcaactgtcctggtgcgccacgtctggagttcatggcgggtcgcccgaataccacgatcccggcagttgaaggtctgattccggagccgcaggacagcgtcaccaaaattctgcagcgtttcgaggatgccggtaactttagcccgttcgaggtcgtgagcctgttggcgagccatacggtggcgcgtgctgacaaagttgatgaaaccatcgacgccgctccgttcgacagcaccccgtttacgtttgatacccaggttttcctggaagttctgttgaaaggcaccggctttccgggttccaataacaacaccggtgaagtcatgtctccgctgcctctgggctcgggtagcgatactggtgagatgcgcctgcaaagcgactttgctctggcccgtgatgagcgtaccgcgtgcttctggcagtccttcgtcaacgaacaagagtttatggcggccagctttaaggctgcgatggcaaaactggcaattctgggccatagccgttccagcctgatcgattgcagcgacgtggttccggtgccgaagcctgcggtcaataagccggcgaccttcccggcgaccaaaggcccgaaggacctggatactctgacgtgtaaagcgctgaagtttccgacgctgacgtctgatccgggtgccacggagactctgatcccgcactgcagcaatggtggcatgagctgcccgggtgtgcaattcgacggtccggcgtaatactagagccaggcatcaaataaaacgaaaggctcagtcgaaagactgggcctttcgttttatctgttgtttgtcggtgaacgctctctactagagtcacactggctcaccttcgggtgggcctttctgcgtttatagtcgacttgacagctagctcagtcctaggtattgtgctagctactagagaaagaggagaaatactagatgtcccgccctcaattcacctcgctccgtttgtctttgctcgcactcgccgtatccgcaacgctgccgacctttgccttcgctaccgaaaccatgaccgttaccgcgaccggcaacgcacgcagctcgttcgaggcgccgatgatggtgagcgtgatcgatacctctgctccggagaaccagacggcgacgagcgctaccgatctgctgcgccacgtgccgggtattacgctggacggtaccggtcgcacgaacggtcaagacgtgaacatgcgcggctacgaccatcgcggtgtgctggtcctggtcgatggtgtgcgtcagggtacggataccggtcacttgaatggtacctttctggatccggcgctgattaagcgtgtcgaaatcgtgcgtggcccgtcggcactgctgtatggtagcggtgcgctgggcggtgtgatcagctacgataccgtcgatgcgaaagacctgttgcaagagggtcaaagctccggtttccgcgtttttggtactggtggtaccggtgaccatagcctgggcctgggcgcgagcgcgtttggtcgcacggaaaacctggatggcatcgttgcgtggagcagccgtgatcgtggtgacttgcgccagtctaatggcgaaacggcccctaacgatgaaagcattaacaacatgctggccaagggtacgtggcagatcgatagcgcgcagagcctgagcggcctggtccgttactacaacaacgacgcgcgtgagccgaaaaacccgcagacggtcgaggcgagcgagagcagcaacccgatggtggaccgtagcaccattcaacgtgatgcccaactgagctataagctggcaccgcaaggtaatgactggctgaatgcggatgcgaaaatctactggagcgaagttcgcatcaatgcacagaatacgggtagctctggcgagtaccgtgaacagattaccaaaggtgcacgtctggagaatcgttctacgctgtttgctgacagcttcgcttcgcatctgctgacgtatggtggcgagtattatcgtcaggaacaacacccaggtggtgcgaccacgggtttcccgcaggcgaagatcgattttagcagcggctggctgcaagatgagatcaccttgcgtgacttgccgattaccctgctgggtggtacgcgttatgacagctaccgtggcagcagcgacggttacaaagacgtcgatgcagataaatggagctcccgtgccggcatgaccattaatccgaccaattggctgatgctgttcggcagctatgcgcaagcgttccgtgccccaaccatgggtgagatgtacaatgacagcaagcatttcagcattggtcgcttctacacgaattactgggtgccgaacccgaatctgcgtccggagactaatgaaacccaggagtatggttttggcctgcgctttgatgatctgatgctgagcaacgacgccctggaattcaaggcgagctactttgacactaaagccaaagactacattagcactacggttgattttgcggctgctaccaccatgtcctataatgttccaaacgcaaagatttggggctgggacgtcatgaccaagtacaccaccgacctgtttagcttggatgttgcatacaatcgcacccgtggcaaagacaccgataccggcgaatacatcagcagcatcaatccggacaccgttacgtccaccctgaacatcccgattgcgcacagcggtttcagcgttggttgggttggtacgtttgcggatcgctccacccacatctcgtcgtcttatagcaagcaaccgggctacggcgtgaatgatttctatgtgagctatcagggccagcaagccctgaaaggtatgacgactaccctggttctgggcaacgcattcgacaaagagtattggagcccgcagggcattccgcaggacggtcgtaacggcaagattttcgtttcctaccaatggtaaaagcttggctgttttggcggatgagagaagattttcagcctgatacagattaaatcagaacgcagaagcggtctgataaaacagaatttgcctggcggcagtagcgcggtggtcccacctgaccccatgccgaactcagaagtgaaacgccgtagcgccgatggtagtgtggggtctccccatgcgagagtagggaactgccaggcatcaaataaaacgaaaggctcagtcgaaagactgggcctttcgttttatctgttgtttgtcggtgaacgctctcctgagtaggacaaatccgccgggagcggatttgaacgttgcgaagcaacggcccggagggtggcgggcaggacgcccgccataaactgccaggcatcaaattaagcagaaggccatcctgacggatggcctttttgcgtttctacaaactcttttgtttatttttctaaatacattcaaatatgtatccgctcatgagacaataaccctgataaatgcttcaataatattgaaaaaggaagagtatgagtattcaacatttccgtgtcgcccttattcccttttttgcggcattttgccttcctgtttttgctcacccagaaacgctggtgaaagtaaaagatgctgaagatcagttgggtgcacgagtgggttacatcgaactggatctcaacagcggtaagatccttgagagttttcgccccgaagaacgttttccaatgatgagcacttttaaagttctgctatgtggcgcggtattatcccgtgttgacgccgggcaagagcaactcggtcgccgcatacactattctcagaatgacttggttgagtactcaccagtcacagaaaagcatcttacggatggcatgacagtaagagaattatgcagtgctgccataaccatgagtgataacactgcggccaacttacttctgacaacgatcggaggaccgaaggagctaaccgcttttttgcacaacatgggggatcatgtaactcgccttgatcgttgggaaccggagctgaatgaagccataccaaacgacgagcgtgacaccacgatgcctgtagcaatggcaacaacgttgcgcaaactattaactggcgaactacttactctagcttcccggcaacaattaatagactggatggaggcggataaagttgcaggaccacttctgcgctcggcccttccggctggctggtttattgctgataaatctggagccggtgagcgtgggtctcgcggtatcattgcagcactggggccagatggtaagccctcccgtatcgtagttatctacacgacggggagtcaggcaactatggatgaacgaaatagacagatcgctgagataggtgcctcactgattaagcattggtaactgtcagaccaagtttactcatatatactttagattgatttacgcgccctgtagcggcgcattaagcgcggcgggtgtggtggttacgcgcagcgtgaccgctacacttgccagcgccctagcgcccgctcctttcgctttcttcccttcctttctcgccacgttcgccggctttccccgtcaagctctaaatcgggggctccctttagggttccgatttagtgctttacggcacctcgaccccaaaaaacttgatttgggtgatggttcacgtagtgggccatcgccctgatagacggtttttcgccctttgacgttggagtccacgttctttaatagtggactcttgttccaaacttgaacaacactcaaccctatctcgggctattcttttgatttataagggattttgccgatttcggcctattggttaaaaaatgagctgatttaacaaaaatttaacgcgaattttaacaaaatattaacgtttacaatttaaaaggatctaggtgaagatcctttttgataatctcatgaccaaaatcccttaacgtgagttttcgttccactgagcgtcagaccccgtagaaaagatcaaaggatcttcttgagatcctttttttctgcgcgtaatctgctgcttgcaaacaaaaaaaccaccgctaccagcggtggtttgtttgccggatcaagagctaccaactctttttccgaaggtaactggcttcagcagagcgcagataccaaatactgtccttctagtgtagccgtagttaggccaccacttcaagaactctgtagcaccgcctacatacctcgctctgctaatcctgttaccagtggctgctgccagtggcgataagtcgtgtcttaccgggttggactcaagacgatagttaccggataaggcgcagcggtcgggctgaacggggggttcgtgcacacagcccagcttggagcgaacgacctacaccgaactgagatacctacagcgtgagctatgagaaagcgccacgcttcccgaagggagaaaggcggacaggtatccggtaagcggcagggtcggaacaggagagcgcacgagggagcttccagggggaaacgcctggtatctttatagtcctgtcgggtttcgccacctctgacttgagcgtcgatttttgtgatgctcgtcaggggggcggagcctatggaaaaacgccagcaacgcggcctttttacggttcctggccttttgctggccttttgctcacatgttctttcctgcgttatcccctgattctgtggataaccgtattaccgcctttgagtgagctgataccgctcgccgcagccgaacgaccgagcgcagcgagtcagtgagcgaggaagcggaagagcgcctgatgcggtattttctccttacgcatctgtgcggtatttcacaccgcatagggtcatggctgcgccccgacacccgccaacacccgctgacgcgccctgacgggcttgtctgctcccggcatccgcttacagacaagctgtgaccgtctccgggagctgcatgtgtcagaggttttcaccgtcatcaccgaaacgcgcgaggcagcaaggagatggcgcccaacagtcccccggccacggggcctgccaccatacccacgccgaaacaagcgctcatgagcccgaagtggcgagcccgatcttccccatcggtgatgtcggcgatataggcgccagcaaccgcacctgtggcgccggtgatgccggccacgatgcgtccggcgtagaggatctgctcatgtttgacagcttatc

SEQ ID NO: 29 - DNA, 7316 bp, Artificial Sequence
  pPRO33-PDI expression construct
atcgattcagcttttcagccgccgccagaacgtcgtccggctgatgcctaaataattcgccgctgctgttttatcgccattaaatttctccagtgcctgttgtggtgtcagtaagcgtggagcgggagttttcgccgactcgcgcgccagttccggcagtagcagttgcataaactgcggcgttaaatccggcgtcggttccacacttaaaaacagcgccagtcgttccatcatattgcgcagttcacgaatattgcctggccagtcgtagtgcagcagcacagtttcacttgcctgtaacccctggcgtaatgcagcagaaaatggggcggagagcgccgccagagacactttcaaaaagctttccgccagcggaagaatatccgccacccgctcgcgcagtggtggcaattgcagacgcaaaatactcagccgataaaacagatcacggcgaaaacgtccttgctgcatatcttcttccagattgcagtgagtggcgctaatgacccgtacatctaccggaacaggctgatgcccgccgacgcgggtgacctctttttcttccagcacccgcagcagccgggtctgcaaaggtagcggcatttcgccaatctcatccagaaacagcgtaccgccgtgggcaatttcgaacagcccggcgcgacctccgcgtcgcgagccggtaaacgccccttcctcatagccaaacagttctgcttccagcagcgattcggcaatcgccccgcagttgacggcaacaaacggatgcgactttttgccctgtcgcgcatcgtggcgggcaaaatattcccgatgaatcgcctgggccgccagctctttgcccgtccccgtttccccctcaatcaacaccgccgcactggagcgggcatacagcaaaatagtctgccgtacttgttccatctgtggtgattgaccgagcatatcgcccagcacgtaacgagtacgcagggcgttgcgggtggcatcgtgagtgttatggcgtaacgacatgcgcgtcatatccagcgcatcgctgaacgcctggcgcacggtggcggcggaatagataaaaattccggtcattccggcttcttctgccaaatcggtaatcagccctgcgccgaccaccgcttcggtgccgttagcttttagctcgttaatctgcccgcgtgcgtcttcctcggtaatgtagctacgttggtcgaggcgcaaattaaaggttttttgaaacgccaccagcgctggaatggtttcctgataggtgacaacgccgatagaagaggtgagttttccggcttttgccagtgcctgtaacacatcgtagccgctcggtttaatcaaaataactggcactgacaggcggcttttcaggtacgcgccgttagagccagccgcgatgatggcgtcacagcgttcgtttgccagtttcttgcggatgtaggtcactgctttttcaaagccaagctgaataggggtaatgttcgccaggtgatcaaactcgaggctgatatcgcgaaacagctcgaacaggcgcgttacagataccgtccagataaccggtttgtcgtcattaagccgtggtggatgtgccatagcgcaccgcaaagttaagaaaccgaatattgggtttagtcttgtttcataattgttgcaatgaaacgcggtgaaacattgcctgaaacgttaactgaaacgcatatttgcggattagttcatgactttatctctaacaaattgaaattaaacatttaattttattaaggcaattgtggcacaccccttgctttgtctttatcaacgcaaataacaagttgataacaagctagcaggaggaattcaccatgtctgatgttgtacaactgaagaaagatacgttcgatgactttatcaaaactaatgacttggtgctggcagagtttttcgccccgtggtgtggccactgcaaagctctggctccggagtacgaagaggccgcgaccaccctgaaagaaaagaacatcaaactggcgaaagtggactgtacggaagaaaccgacctgtgtcagcagcacggcgtggaaggttacccgaccctgaaggtgtttcgtggcctggacaatgttagcccgtacaaaggtcaacgtaaggccgcagcgatcaccagctacatgatcaagcagtcgctgcctgcagtctctgaggtgaccaaagataatctggaagagttcaaaaaggcagataaggcggtgctggttgcctatgttgatgcaagcgacaaggcgagcagcgaggtctttacccaggtcgcggagaaattgcgcgataactacccgttcggcagcagctccgatgcagctttggccgaggcggaaggtgtcaaggctccggcgatcgttctgtacaaagatttcgacgagggtaaagcggtgttcagcgaaaagtttgaggtggaagcaattgaaaagttcgcaaaaaccggtgccacgcctttgattggcgaaatcggtccggaaacctattctgactatatgagcgccggtatcccgctggcctacattttcgcagaaacggcagaagagcgcaaagaactgagcgacaagttgaagccaattgcagaggcacagcgtggcgtcatcaactttggtaccattgacgcgaaagcatttggtgcgcatgccggtaacctgaatctgaaaacggacaaatttccggcgtttgcgattcaagaggtggcgaagaaccaaaagtttccgttcgatcaagaaaaagagattaccttcgaggcgatcaaagcgttcgttgacgactttgttgccggtaaaatcgagccgagcattaagagcgagccgatcccggagaagcaggaaggcccggtgaccgtcgtcgtcgcgaagaattacaacgagattgttctggatgacacgaaagacgtcctgattgagttctatgcgccgtggtgcggtcattgcaaagcgctggccccgaaatatgaagagctgggtgcgctgtacgcgaagagcgagtttaaggaccgtgtggttatcgcgaaagtagatgcgaccgccaatgacgttcctgacgagatccaaggcttcccgaccattaaactgtatccggctggtgctaaaggccagccagttacctatagcggtagccgcacggttgaggatctgattaagttcattgccgagaacggcaagtacaaggcggcaatcagcgaggatgcagaagaaacgagctccgcaaccgaaaccacgacggaaaccgctactaagtccgaagaggcggcgaaagaaaccgcgacggagcacgatgagctgtaagtcgacctgcaggcatgcaagcttggctgttttggcggatgagagaagattttcagcctgatacagattaaatcagaacgcagaagcggtctgataaaacagaatttgcctggcggcagtagcgcggtggtcccacctgaccccatgccgaactcagaagtgaaacgccgtagcgccgatggtagtgtggggtctccccatgcgagagtagggaactgccaggcatcaaataaaacgaaaggctcagtcgaaagactgggcctttcgttttatctgttgtttgtcggtgaacgctctcctgagtaggacaaatccgccgggagcggatttgaacgttgcgaagcaacggcccggagggtggcgggcaggacgcccgccataaactgccaggcatcaaattaagcagaaggccatcctgacggatggcctttttgcgtttctacaaactcttttgtttatttttctaaatacattcaaatatgtatccgctcatgagacaataaccctgataaatgcttcaataatattgaaaaaggaagagtatgagtattcaacatttccgtgtcgcccttattcccttttttgcggcattttgccttcctgtttttgctcacccagaaacgctggtgaaagtaaaagatgctgaagatcagttggggcaaactattaactggcgaactacttactctagcttcccggcaacaattaatagactggatggaggcggataaagttgcaggaccacttctgcgctcggcccttccggctggctggtttattgctgataaatctggagccggtgagcgtgggtctcgcggtatcattgcagcactggggccagatggtaagccctcccgtatcgtagttatctacacgacggggagtcaggcaactatggatgaacgaaatagacagatcgctgagataggtgcctcactgattaagcattggtaactgtcagaccaagtttactcatatatactttagattgatttacgcgccctgtagcggcgcattaagcgcggcgggtgtggtggttacgcgcagcgtgaccgctacacttgccagcgccctagcgcccgctcctttcgctttcttcccttcctttctcgccacgttcgccggctttccccgtcaagctctaaatcgggggctccctttagggttccgatttagtgctttacggcacctcgaccccaaaaaacttgatttgggtgatggttcacgtagtgggccatcgccctgatagacggtttttcgccctttgacgttggagtccacgttctttaatagtggactcttgttccaaacttgaacaacactcaaccctatctcgggctattcttttgatttataagggattttgccgatttcggcctattggttaaaaaatgagctgatttaacaaaaatttaacgcgaattttaacaaaatattaacgtttacaatttaaaaggatctaggtgaagatcctttttgataatctcatgaccaaaatcccttaacgtgagttttcgttccactgagcgtcagaccccgtagaaaagatcaaaggatcttcttgagatcctttttttctgcgcgtaatctgctgcttgcaaacaaaaaaaccaccgctaccagcggtggtttgtttgccggatcaagagctaccaactctttttccgaaggtaactggcttcagcagagcgcagataccaaatactgtccttctagtgtagccgtagttaggccaccacttcaagaactctgtagcaccgcctacatacctcgctctgctaatcctgttaccagtcaggcatttgagaagcacacggtcacactgcttccggtagtcaataaaccggtaaaccagcaatagacataagcggctatttaacgaccctgccctgaaccgacgaccgggtcgaatttgctttcgaatttctgccattcatccgcttattatcacttattcaggcgtagcaccaggcgtttaagggcaccaataactgccttaaaaaaattacgccccgccctgccactcatcgcagtactgttgtaattcattaagcattctgccgacatggaagccatcacagacggcatgatgaacctgaatcgccagcggcatcagcaccttgtcgccttgcgtataatatttgcccatggtgaaaacgggggcgaagaagttgtccatattggccacgtttaaatcaaaactggtgaaactcacccagggattggctgagacgaaaaacatattctcaataaaccctttagggaaataggccaggttttcaccgtaacacgccacatcttgcgaatatatgtgtagaaactgccggaaatcgtcgtggtattcactccagagcgatgaaaacgtttcagtttgctcatggaaaacggtgtaacaagggtgaacactatcccatatcaccagctcaccgtctttcattgccatacggaattccggatgagcattcatcaggcgggcaagaatgtgaataaaggccggataaaacttgtgcttatttttctttacggtctttaaaaaggccgtaatatccagctgaacggtctggttataggtacattgagcaactgactgaaatgcctcaaaatgttctttacgatgccattgggatatatcaacggtggtatatccagtgatttttttctccattttagcttccttagctcctgaaaatctcgataactcaaaaaatacgcccggtagtgatcttatttcattatggtgaaagttggaacctcttacgtgccgatcaacgtctcattttcgccaaaagttggcccagggcttcccggtatcaacagggacaccaggatttatttattctgcgaagtgatcttccgtcacaggtatttattcggcgcaaagtgcgtcgggtgatgctgccaacttactgatttagtgtatgatggtgtttttgaggtgctccagtggcttctgtttctatcagctgtccctcctgttcagctactgacggggtggtgcgtaacggcaaaagcaccgccggacatcagcgctagcggagtgtatactggcttactatgttggcactgatgagggtgtcagtgaagtgcttcatgtggcaggagaaaaaaggctgcaccggtgcgtcagcagaatatgtgatacaggatatattccgcttcctcgctcactgactcgctacgctcggtcgttcgactgcggcgagcggaaatggcttacgaacggggcggagatttcctggaagatgccaggaagatacttaacagggaagtgagagggccgcggcaaagccgtttttccataggctccgcccccctgacaagcatcacgaaatctgacgctcaaatcagtggtggcgaaacccgacaggactataaagataccaggcgtttccccctggcggctccctcgtgcgctctcctgttcctgcctttcggtttaccggtgtcattccgctgttatggccgcgtttgtctcattccacgcctgacactcagttccgggtaggcagttcgctccaagctggactgtatgcacgaaccccccgttcagtccgaccgctgcgccttatccggtaactatcgtcttgagtccaacccggaaagacatgcaaaagcaccactggcagcagccactggtaattgatttagaggagttagtcttgaagtcatgcgccggttaaggctaaactgaaaggacaagttttggtgactgcgctcctccaagccagttacctcggttcaaagagttggtagctcagagaaccttcgaaaaaccgccctgcaaggcggttttttcgttttcagagcaagagattacgcgcagaccaaaacgatctcaagaagatcatcttattaatcagataaaatatttgctcatgagcccgaagtggcgagcccgatcttccccatcggtgatgtcggcgatataggcgccagcaaccgcacctgtggcgccggtgatgccggccacgatgcgtccggcgtagaggatctgctcatgtttgacagcttatc

SEQ ID NO: 30 - protein, 451 aa, Artificial Sequence
  Infliximab chimeric (murine variable doman, human constant domain) heavy chain
MEVKLEESGGGLVQPGGSMKLSCVASGFIFSNHWMNWVRQSPEKGLEWVAEIRSKSINSATHYAESVKGRFTISRDDSKSAVYLQMTDLRTEDTGVYYCSRNYYGSTYDYWGQGTTLTVSSASTKGPSVFPLAPSSKSTSGGTAALGCLVKDYFPEPVTVSWNSGALTSGVHTFPAVLQSSGLYSLSSVVTVPSSSLGTQTYICNVNHKPSNTKVDKKVEPKSCDKTHTCPPCPAPELLGGPSVFLFPPKPKDTLMISRTPEVTCVVVDVSHEDPEVKFNWYVDGVEVHNAKTKPREEQYNSTYRVVSVLTVLHQDWLNGKEYKCKVSNKALPAPIEKTISKAKGQPREPQVYTLPPSRDELTKNQVSLTCLVKGFYPSDIAVEWESNGQPENNYKTTPPVLDSDGSFFLYSKLTVDKSRWQQGNVFSCSVMHEALHNHYTQKSLSLSPGK

SEQ ID NO: 31 - protein, 215 aa, Artificial Sequence
  Infliximab chimeric (murine variable doman, human constant domain) light chain
MDILLTQSPAILSVSPGERVSFSCRASQFVGSSIHWYQQRTNGSPRLLIKYASESMSGIPSRFSGSGSGTDFTLSINTVESEDIADYYCQQSHSWPFTFGSGTNLEVKRTVAAPSVFIFPPSDEQLKSGTASVVCLLNNFYPREAKVQWKVDNALQSGNSQESVTEQDSKDSTYSLSSTLTLSKADYEKHKVYACEVTHQGLSSPVTKSFNRGEC

SEQ ID NO: 32 - DNA, 5875 bp, Artificial Sequence
  pBAD24-Infliximab_HC expression construct
atcgatgcataatgtgcctgtcaaatggacgaagcagggattctgcaaaccctatgctactccgtcaagccgtcaattgtctgattcgttaccaattatgacaacttgacggctacatcattcactttttcttcacaaccggcacggaactcgctcgggctggccccggtgcattttttaaatacccgcgagaaatagagttgatcgtcaaaaccaacattgcgaccgacggtggcgataggcatccgggtggtgctcaaaagcagcttcgcctggctgatacgttggtcctcgcgccagcttaagacgctaatccctaactgctggcggaaaagatgtgacagacgcgacggcgacaagcaaacatgctgtgcgacgctggcgatatcaaaattgctgtctgccaggtgatcgctgatgtactgacaagcctcgcgtacccgattatccatcggtggatggagcgactcgttaatcgcttccatgcgccgcagtaacaattgctcaagcagatttatcgccagcagctccgaatagcgcccttccccttgcccggcgttaatgatttgcccaaacaggtcgctgaaatgcggctggtgcgcttcatccgggcgaaagaaccccgtattggcaaatattgacggccagttaagccattcatgccagtaggcgcgcggacgaaagtaaacccactggtgataccattcgcgagcctccggatgacgaccgtagtgatgaatctctcctggcgggaacagcaaaatatcacccggtcggcaaacaaattctcgtccctgatttttcaccaccccctgaccgcgaatggtgagattgagaatataacctttcattcccagcggtcggtcgataaaaaaatcgagataaccgttggcctcaatcggcgttaaacccgccaccagatgggcattaaacgagtatcccggcagcaggggatcattttgcgcttcagccatacttttcatactcccgccattcagagaagaaaccaattgtccatattgcatcagacattgccgtcactgcgtcttttactggctcttctcgctaaccaaaccggtaaccccgcttattaaaagcattctgtaacaaagcgggaccaaagccatgacaaaaacgcgtaacaaaagtgtctataatcacggcagaaaagtccacattgattatttgcacggcgtcacactttgctatgccatagcatttttatccataagattagcggatcctacctgacgctttttatcgcaactctctactgtttctccatacccgtttttttgggctagcaggaggaattcaccatggaagttaaattagaagaaagcggcggcggtttggtgcaacctggcggttcgatgaagttgagctgcgtcgcaagcggtttcattttttccaaccactggatgaactgggtgcgccagtctccggaaaagggtctggaatgggttgcggagatccgtagcaagagcatcaatagcgcgacgcattatgccgagagcgtcaaaggccgcttcaccatttctcgtgacgacagcaaaagcgctgtgtatctgcaaatgaccgacttgcgtaccgaggacacgggcgtgtattactgctcccgcaactattacggttccacctacgactactggggccagggtacgaccctgaccgttagctcggcgagcaccaagggtccgagcgtctttccgctggcaccgagcagcaaaagcaccagcggtggtaccgccgcactgggttgcctggtgaaagattacttcccggaaccggttactgtgagctggaacagcggcgcgctgacctctggcgtgcacacgttcccggcagttctgcaaagcagcggcctgtactccctgtccagcgtcgtcaccgtgccgagcagcagcctgggtacgcaaacctatatttgtaacgtcaatcacaagccgagcaacaccaaagtggacaaaaaagtcgaaccgaaaagctgcgataaaacccatacttgtccgccgtgcccggccccggagcttctgggtggtccaagcgtttttctgttcccgccgaagccgaaagacaccctgatgatcagccgcacccctgaggtgacctgtgtggtagttgacgtttcccacgaagatccagaggtcaagtttaactggtatgtggatggcgtcgaagttcacaatgcaaagaccaagccgcgtgaagaacagtataactctacgtaccgtgtcgtgagcgttctgactgttctgcaccaggattggctgaacggcaaagagtacaagtgcaaggttagcaataaagcgctgccggctccgatcgagaaaaccatttctaaggctaaaggtcagccgcgtgagccgcaagtttacaccctgccaccgagccgtgatgagctgacgaaaaatcaagtatctctgacctgtctggtcaaaggtttttacccaagcgatatcgcggttgaatgggagagcaacggccagccggagaataattacaagacgacgcctccggtgctggatagcgatggttcgtttttcctgtacagcaagttgacggttgataaaagccgttggcaacagggtaacgtgttctcctgttccgtcatgcatgaagcgctgcacaaccattatactcagaaaagcctcagcctgtccccgggtaaataagtcgacctgcaggcatgcaagcttggctgttttggcggatgagagaagattttcagcctgatacagattaaatcagaacgcagaagcggtctgataaaacagaatttgcctggcggcagtagcgcggtggtcccacctgaccccatgccgaactcagaagtgaaacgccgtagcgccgatggtagtgtggggtctccccatgcgagagtagggaactgccaggcatcaaataaaacgaaaggctcagtcgaaagactgggcctttcgttttatctgttgtttgtcggtgaacgctctcctgagtaggacaaatccgccgggagcggatttgaacgttgcgaagcaacggcccggagggtggcgggcaggacgcccgccataaactgccaggcatcaaattaagcagaaggccatcctgacggatggcctttttgcgtttctacaaactcttttgtttatttttctaaatacattcaaatatgtatccgctcatgagacaataaccctgataaatgcttcaataatattgaaaaaggaagagtatgagtattcaacatttccgtgtcgcccttattcccttttttgcggcattttgccttcctgtttttgctcacccagaaacgctggtgaaagtaaaagatgctgaagatcagttgggtgcacgagtgggttacatcgaactggatctcaacagcggtaagatccttgagagttttcgccccgaagaacgttttccaatgatgagcacttttaaagttctgctatgtggcgcggtattatcccgtgttgacgccgggcaagagcaactcggtcgccgcatacactattctcagaatgacttggttgagtactcaccagtcacagaaaagcatcttacggatggcatgacagtaagagaattatgcagtgctgccataaccatgagtgataacactgcggccaacttacttctgacaacgatcggaggaccgaaggagctaaccgcttttttgcacaacatgggggatcatgtaactcgccttgatcgttgggaaccggagctgaatgaagccataccaaacgacgagcgtgacaccacgatgcctgtagcaatggcaacaacgttgcgcaaactattaactggcgaactacttactctagcttcccggcaacaattaatagactggatggaggcggataaagttgcaggaccacttctgcgctcggcccttccggctggctggtttattgctgataaatctggagccggtgagcgtgggtctcgcggtatcattgcagcactggggccagatggtaagccctcccgtatcgtagttatctacacgacggggagtcaggcaactatggatgaacgaaatagacagatcgctgagataggtgcctcactgattaagcattggtaactgtcagaccaagtttactcatatatactttagattgatttacgcgccctgtagcggcgcattaagcgcggcgggtgtggtggttacgcgcagcgtgaccgctacacttgccagcgccctagcgcccgctcctttcgctttcttcccttcctttctcgccacgttcgccggctttccccgtcaagctctaaatcgggggctccctttagggttccgatttagtgctttacggcacctcgaccccaaaaaacttgatttgggtgatggttcacgtagtgggccatcgccctgatagacggtttttcgccctttgacgttggagtccacgttctttaatagtggactcttgttccaaacttgaacaacactcaaccctatctcgggctattcttttgatttataagggattttgccgatttcggcctattggttaaaaaatgagctgatttaacaaaaatttaacgcgaattttaacaaaatattaacgtttacaatttaaaaggatctaggtgaagatcctttttgataatctcatgaccaaaatcccttaacgtgagttttcgttccactgagcgtcagaccccgtagaaaagatcaaaggatcttcttgagatcctttttttctgcgcgtaatctgctgcttgcaaacaaaaaaaccaccgctaccagcggtggtttgtttgccggatcaagagctaccaactctttttccgaaggtaactggcttcagcagagcgcagataccaaatactgtccttctagtgtagccgtagttaggccaccacttcaagaactctgtagcaccgcctacatacctcgctctgctaatcctgttaccagtggctgctgccagtggcgataagtcgtgtcttaccgggttggactcaagacgatagttaccggataaggcgcagcggtcgggctgaacggggggttcgtgcacacagcccagcttggagcgaacgacctacaccgaactgagatacctacagcgtgagctatgagaaagcgccacgcttcccgaagggagaaaggcggacaggtatccggtaagcggcagggtcggaacaggagagcgcacgagggagcttccagggggaaacgcctggtatctttatagtcctgtcgggtttcgccacctctgacttgagcgtcgatttttgtgatgctcgtcaggggggcggagcctatggaaaaacgccagcaacgcggcctttttacggttcctggccttttgctggccttttgctcacatgttctttcctgcgttatcccctgattctgtggataaccgtattaccgcctttgagtgagctgataccgctcgccgcagccgaacgaccgagcgcagcgagtcagtgagcgaggaagcggaagagcgcctgatgcggtattttctccttacgcatctgtgcggtatttcacaccgcatagggtcatggctgcgccccgacacccgccaacacccgctgacgcgccctgacgggcttgtctgctcccggcatccgcttacagacaagctgtgaccgtctccgggagctgcatgtgtcagaggttttcaccgtcatcaccgaaacgcgcgaggcagcaaggagatggcgcccaacagtcccccggccacggggcctgccaccatacccacgccgaaacaagcgctcatgagcccgaagtggcgagcccgatcttccccatcggtgatgtcggcgatataggcgccagcaaccgcacctgtggcgccggtgatgccggccacgatgcgtccggcgtagaggatctgctcatgtttgacagcttatc

SEQ ID NO: 33 - DNA, 6503 bp, Artificial Sequence
  pPRO33-Infliximab_LC expression construct
atcgattcagcttttcagccgccgccagaacgtcgtccggctgatgcctaaataattcgccgctgctgttttatcgccattaaatttctccagtgcctgttgtggtgtcagtaagcgtggagcgggagttttcgccgactcgcgcgccagttccggcagtagcagttgcataaactgcggcgttaaatccggcgtcggttccacacttaaaaacagcgccagtcgttccatcatattgcgcagttcacgaatattgcctggccagtcgtagtgcagcagcacagtttcacttgcctgtaacccctggcgtaatgcagcagaaaatggggcggagagcgccgccagagacactttcaaaaagctttccgccagcggaagaatatccgccacccgctcgcgcagtggtggcaattgcagacgcaaaatactcagccgataaaacagatcacggcgaaaacgtccttgctgcatatcttcttccagattgcagtgagtggcgctaatgacccgtacatctaccggaacaggctgatgcccgccgacgcgggtgacctctttttcttccagcacccgcagcagccgggtctgcaaaggtagcggcatttcgccaatctcatccagaaacagcgtaccgccgtgggcaatttcgaacagcccggcgcgacctccgcgtcgcgagccggtaaacgccccttcctcatagccaaacagttctgcttccagcagcgattcggcaatcgccccgcagttgacggcaacaaacggatgcgactttttgccctgtcgcgcatcgtggcgggcaaaatattcccgatgaatcgcctgggccgccagctctttgcccgtccccgtttccccctcaatcaacaccgccgcactggagcgggcatacagcaaaatagtctgccgtacttgttccatctgtggtgattgaccgagcatatcgcccagcacgtaacgagtacgcagggcgttgcgggtggcatcgtgagtgttatggcgtaacgacatgcgcgtcatatccagcgcatcgctgaacgcctggcgcacggtggcggcggaatagataaaaattccggtcattccggcttcttctgccaaatcggtaatcagccctgcgccgaccaccgcttcggtgccgttagcttttagctcgttaatctgcccgcgtgcgtcttcctcggtaatgtagctacgttggtcgaggcgcaaattaaaggttttttgaaacgccaccagcgctggaatggtttcctgataggtgacaacgccgatagaagaggtgagttttccggcttttgccagtgcctgtaacacatcgtagccgctcggtttaatcaaaataactggcactgacaggcggcttttcaggtacgcgccgttagagccagccgcgatgatggcgtcacagcgttcgtttgccagtttcttgcggatgtaggtcactgctttttcaaagccaagctgaataggggtaatgttcgccaggtgatcaaactcgaggctgatatcgcgaaacagctcgaacaggcgcgttacagataccgtccagataaccggtttgtcgtcattaagccgtggtggatgtgccatagcgcaccgcaaagttaagaaaccgaatattgggtttagtcttgtttcataattgttgcaatgaaacgcggtgaaacattgcctgaaacgttaactgaaacgcatatttgcggattagttcatgactttatctctaacaaattgaaattaaacatttaattttattaaggcaattgtggcacaccccttgctttgtctttatcaacgcaaataacaagttgataacaagctagcaggaggaattcaccatggatattttattgacccaaagcccagccattctgtctgtttccccgggcgagcgtgtttcttttagctgccgtgcaagccagttcgttggttcatcgatccactggtaccaacagcgtacgaacggtagcccgcgtctgctgattaagtacgcgagcgaaagcatgagcggtatcccgagccgcttcagcggtagcggcagcggcacggacttcacgctgagcatcaatacggttgaaagcgaggacatcgcggactattactgccagcagagccattcttggccgtttacctttggcagcggtaccaatctggaagttaaacgcaccgtggcagcgccgtccgttttcatttttcctccgtccgatgagcaactgaaatcgggcacggccagcgtcgtgtgtctgttgaacaacttctacccgcgtgaggcgaaggtgcagtggaaagtggacaacgcgctgcaatccggtaatagccaggaaagcgtcaccgaacaagatagcaaggacagcacctacagcctgagctctactctgaccctgagcaaggctgattatgagaaacacaaggtctatgcatgtgaggtgacccatcagggtctgtccagcccggtcaccaaaagcttcaatcgcggtgagtgctaagtcgacctgcaggcatgcaagcttggctgttttggcggatgagagaagattttcagcctgatacagattaaatcagaacgcagaagcggtctgataaaacagaatttgcctggcggcagtagcgcggtggtcccacctgaccccatgccgaactcagaagtgaaacgccgtagcgccgatggtagtgtggggtctccccatgcgagagtagggaactgccaggcatcaaataaaacgaaaggctcagtcgaaagactgggcctttcgttttatctgttgtttgtcggtgaacgctctcctgagtaggacaaatccgccgggagcggatttgaacgttgcgaagcaacggcccggagggtggcgggcaggacgcccgccataaactgccaggcatcaaattaagcagaaggccatcctgacggatggcctttttgcgtttctacaaactcttttgtttatttttctaaatacattcaaatatgtatccgctcatgagacaataaccctgataaatgcttcaataatattgaaaaaggaagagtatgagtattcaacatttccgtgtcgcccttattcccttttttgcggcattttgccttcctgtttttgctcacccagaaacgctggtgaaagtaaaagatgctgaagatcagttggggcaaactattaactggcgaactacttactctagcttcccggcaacaattaatagactggatggaggcggataaagttgcaggaccacttctgcgctcggcccttccggctggctggtttattgctgataaatctggagccggtgagcgtgggtctcgcggtatcattgcagcactggggccagatggtaagccctcccgtatcgtagttatctacacgacggggagtcaggcaactatggatgaacgaaatagacagatcgctgagataggtgcctcactgattaagcattggtaactgtcagaccaagtttactcatatatactttagattgatttacgcgccctgtagcggcgcattaagcgcggcgggtgtggtggttacgcgcagcgtgaccgctacacttgccagcgccctagcgcccgctcctttcgctttcttcccttcctttctcgccacgttcgccggctttccccgtcaagctctaaatcgggggctccctttagggttccgatttagtgctttacggcacctcgaccccaaaaaacttgatttgggtgatggttcacgtagtgggccatcgccctgatagacggtttttcgccctttgacgttggagtccacgttctttaatagtggactcttgttccaaacttgaacaacactcaaccctatctcgggctattcttttgatttataagggattttgccgatttcggcctattggttaaaaaatgagctgatttaacaaaaatttaacgcgaattttaacaaaatattaacgtttacaatttaaaaggatctaggtgaagatcctttttgataatctcatgaccaaaatcccttaacgtgagttttcgttccactgagcgtcagaccccgtagaaaagatcaaaggatcttcttgagatcctttttttctgcgcgtaatctgctgcttgcaaacaaaaaaaccaccgctaccagcggtggtttgtttgccggatcaagagctaccaactctttttccgaaggtaactggcttcagcagagcgcagataccaaatactgtccttctagtgtagccgtagttaggccaccacttcaagaactctgtagcaccgcctacatacctcgctctgctaatcctgttaccagtcaggcatttgagaagcacacggtcacactgcttccggtagtcaataaaccggtaaaccagcaatagacataagcggctatttaacgaccctgccctgaaccgacgaccgggtcgaatttgctttcgaatttctgccattcatccgcttattatcacttattcaggcgtagcaccaggcgtttaagggcaccaataactgccttaaaaaaattacgccccgccctgccactcatcgcagtactgttgtaattcattaagcattctgccgacatggaagccatcacagacggcatgatgaacctgaatcgccagcggcatcagcaccttgtcgccttgcgtataatatttgcccatggtgaaaacgggggcgaagaagttgtccatattggccacgtttaaatcaaaactggtgaaactcacccagggattggctgagacgaaaaacatattctcaataaaccctttagggaaataggccaggttttcaccgtaacacgccacatcttgcgaatatatgtgtagaaactgccggaaatcgtcgtggtattcactccagagcgatgaaaacgtttcagtttgctcatggaaaacggtgtaacaagggtgaacactatcccatatcaccagctcaccgtctttcattgccatacggaattccggatgagcattcatcaggcgggcaagaatgtgaataaaggccggataaaacttgtgcttatttttctttacggtctttaaaaaggccgtaatatccagctgaacggtctggttataggtacattgagcaactgactgaaatgcctcaaaatgttctttacgatgccattgggatatatcaacggtggtatatccagtgatttttttctccattttagcttccttagctcctgaaaatctcgataactcaaaaaatacgcccggtagtgatcttatttcattatggtgaaagttggaacctcttacgtgccgatcaacgtctcattttcgccaaaagttggcccagggcttcccggtatcaacagggacaccaggatttatttattctgcgaagtgatcttccgtcacaggtatttattcggcgcaaagtgcgtcgggtgatgctgccaacttactgatttagtgtatgatggtgtttttgaggtgctccagtggcttctgtttctatcagctgtccctcctgttcagctactgacggggtggtgcgtaacggcaaaagcaccgccggacatcagcggtagcggagtgtatactggcttactatgttggcactgatgagggtgtcagtgaagtgcttcatgtggcaggagaaaaaaggctgcaccggtgcgtcagcagaatatgtgatacaggatatattccgcttcctcgctcactgactcgctacgctcggtcgttcgactgcggcgagcggaaatggcttacgaacggggcggagatttcctggaagatgccaggaagatacttaacagggaagtgagagggccgcggcaaagccgtttttccataggctccgcccccctgacaagcatcacgaaatctgacgctcaaatcagtggtggcgaaacccgacaggactataaagataccaggcgtttccccctggcggctccctcgtgcgctctcctgttcctgcctttcggtttaccggtgtcattccgctgttatggccgcgtttgtctcattccacgcctgacactcagttccgggtaggcagttcgctccaagctggactgtatgcacgaaccccccgttcagtccgaccgctgcgccttatccggtaactatcgtcttgagtccaacccggaaagacatgcaaaagcaccactggcagcagccactggtaattgatttagaggagttagtcttgaagtcatgcgccggttaaggctaaactgaaaggacaagttttggtgactgcgctcctccaagccagttacctcggttcaaagagttggtagctcagagaaccttcgaaaaaccgccctgcaaggcggttttttcgttttcagagcaagagattacgcgcagaccaaaacgatctcaagaagatcatcttattaatcagataaaatatttgctcatgagcccgaagtggcgagcccgatcttccccatcggtgatgtcggcgatataggcgccagcaaccgcacctgtggcgccggtgatgccggccacgatgcgtccggcgtagaggatctgctcatgtttgacagcttatc

SEQ ID NO: 34 - DNA, 6545 bp, Artificial Sequence
  pJ1231-03C plasmid
tcagaattggttaattggttgtaacactgacccctatttgtttatttttctaaatacattcaaatatgtatccgctcatgagacaataaccctgataaatgcttcaataatattgaaaaaggaagaatatgagccatattcaacgggaaacgtcgaggccgcgattaaattccaacatggatgctgatttatatgggtataaatgggctcgcgataatgtcgggcaatcaggtgcgacaatctatcgcttgtatgggaagcccgatgcgccagagttgtttctgaaacatggcaaaggtagcgttgccaatgatgttacagatgagatggtcagactaaactggctgacggaatttatgccacttccgaccatcaagcattttatccgtactcctgatgatgcatggttactcaccactgcgatccccggaaaaacagcgttccaggtattagaagaatatcctgattcaggtgaaaatattgttgatgcgctggcagtgttcctgcgccggttgcactcgattcctgtttgtaattgtccttttaacagcgatcgcgtatttcgcctcgctcaggcgcaatcacgaatgaataacggtttggttgatgcgagtgattttgatgacgagcgtaatggctggcctgttgaacaagtctggaaagaaatgcataaacttttgccattctcaccggattcagtcgtcactcatggtgatttctcacttgataaccttatttttgacgaggggaaattaataggttgtattgatgttggacgagtcggaatcgcagaccgataccaggatcttgccatcctatggaactgcctcggtgagttttctccttcattacagaaacggctttttcaaaaatatggtattgataatcctgatatgaataaattgcaatttcatttgatgctcgatgagtttttctaactcatgaccaaaatcccttaacgtgagttacgcgcgcgtcgttccactgagcgtcagaccccgtagaaaagatcaaaggatcttcttgagatcctttttttctgcgcgtaatctgctgcttgcaaacaaaaaaaccaccgctaccagcggtggtttgtttgccggatcaagagctaccaactctttttccgaaggtaactggcttcagcagagcgcagataccaaatactgttcttctagtgtagccgtagttagcccaccacttcaagaactctgtagcaccgcctacatacctcgctctgctaatcctgttaccagtggctgctgccagtggcgataagtcgtgtcttaccgggttggactcaagacgatagttaccggataaggcgcagcggtcgggctgaacggggggttcgtgcacacagcccagcttggagcgaacgacctacaccgaactgagatacctacagcgtgagctatgagaaagcgccacgcttcccgaagggagaaaggcggacaggtatccggtaagcggcagggtcggaacaggagagcgcacgagggagcttccagggggaaacgcctggtatctttatagtcctgtcgggtttcgccacctctgacttgagcgtcgatttttgtgatgctcgtcaggggggcggagcctatggaaaaacgccagcaacgcggcctttttacggttcctggccttttgctggccttttgctcacatgttctttcctgcgttatcccctgattctgtggataaccgtattaccgcctttgagtgagctgataccgctcggggtcgtgcaggtagtttatcattatcaatactcgccatttcaaagaatacgtaaataattaatagtagtgattttcctaactttatttagtcaaaaaattagccttttaattctgctgtaacccgtacatgcccaaaatagggggcgggttacacagaatatataacatcgtaggtgtctgggtgaacagtttattcctggcatccactaaatataatggagcccgctttttaagctggcatccagaaaaaaaaagaatcccagcaccaaaatattgttttcttcaccaaccatcagttcataggtccattctcttagcgcaactacagagaacaggggcacaaacaggcaaaaaacgggcacaacctcaatggagtgatgcaaccagcctggagtaaatgatgacacaaggcaattgacccacgcatgtatctatctcattttcttacaccttctattaccttctgctctctctgatttggaaaaagctgaaaaaaaaggttgaaaccagttccctgaaattattcccctacttgactaataagtatataaagacggtaggtattgattgtaattctgtaaatctatttcttaaacttcttaaattctacttttatagttagtcttttttttagttttaaaacaccagaacttagtttcgacggataaaatgacagctttaactgaaggggccaagcttttcgaaaaagagatcccatatatcaccgaacttgaaggtgacgttgagggtatgaagtttatcataaaaggagaaggcacaggtgatgcgacaacgggtacaatcaaggcaaagtacatttgtacaactggggacctgcctgtcccatgggccactttggtgtctactttgtcttacggcgtacaatgttttgctaagtacccttcacacatcaaagatttctttaagtctgcaatgcctgaaggatacacacaggaacgtacaatttcatttgagggcgacggtgtctataaaacaagagctatggttacttatgaaagaggttccatctacaacagagtgacactaacgggcgaaaatttcaaaaaggatggacatattttgcgtaaaaacgtagctttccaatgcccaccatcaatactatacattctgccagatactgtaaacaatggtattagagtcgagtttaatcaagcttatgatatagaaggtgtcactgaaaaattggttacaaaatgcagccaaatgaatagaccattggcaggatctgccgctgtgcatatccctagataccatcacattacctaccacaccaaattaagtaaagacagggatgaacgaagagatcatatgtgtttagttgaggttgttaaggcagttgatctcgacacttaccaataaatcatgtaattagttatgtcacgcttacattcacgccctccccccacatccgctctaaccgaaaaggaaggagttagacaacctgaagtctaggtccctatttatttttttatagttatgttagtattaagaacgttatttatatttcaaatttttcttttttttctgtacagacgcgtgtacgcatgtaacattatactgaaaaccttgcttgagaaggttttgggacgctcgaaggctttaatttgcggcccctcacctgcacgcaaaataggataattatactctatttctcaacaagtaattggttgtttggccgagcggtctaaggcgcctgattcaagaaatatcttgaccgcagttaactgtgggaatactcaggtatcgtaagatgcaagagttcgaatctcttagcaaccattatttttttcctcaacataacgagaacacacaggggcgctatcgcacagaatcaaattcgatgactggaaattttttgttaatttcagaggtcgcctgacgcatatacctttttcaactgaaaaattgggagaaaaaggaaaggtgagagcgccggaaccggcttttcatatagaatagagaagcgttcatgactaaatgcttgcatcacaatacttgaagttgacaatattatttaaggacctattgttttttccaataggtggttagcaatcgtcttactttctaacttttcttaccttttacatttcagcaatatatatatatatatttcaaggatataccattctaatgtctgcccctaagaagatcgtcgttttgccaggtgaccacgttggtcaagaaatcacagccgaagccattaaggttcttaaagctatttctgatgttcgttccaatgtcaagttcgatttcgaaaatcatttaattggtggtgctgctatcgatgctacaggtgttccacttccagatgaggcgctggaagcctccaagaaggctgatgccgttttgttaggtgctgtgggtggtcctaaatggggtaccggtagtgttagacctgaacaaggtttactaaaaatccgtaaagaacttcaattgtacgccaacttaagaccatgtaactttgcatccgactctcttttagacttatctccaatcaagccacaatttgctaaaggtactgacttcgttgttgtcagagaattagtgggaggtatttactttggtaagagaaaggaagatgatggtgatggtgtcgcttgggatagtgaacaatacaccgttccagaagtgcaaagaatcacaagaatggccgctttcatggccctacaacatgagccaccattgcctatttggtccttggataaagctaatgttttggcctcttcaagattatggagaaaaactgtggaggaaaccatcaagaacgaattccctacattgaaggttcaacatcaattgattgattctgccgccatgatcctagttaagaacccaacccacctaaatggtattataatcaccagcaacatgtttggtgatatcatctccgatgaagcctccgttatcccaggttccttgggtttgttgccatctgcgtccttggcctctttgccagacaagaacaccgcatttggtttgtacgaaccatgccacggttctgctccagatttgccaaagaataaggtcaaccctatcgccactatcttgtctgctgcaatgatgttgaaattgtcattgaacttgcctgaagaaggtaaggccattgaagatgcagttaaaaaggttttggatgcaggcatcagaactggtgatttaggtggttccaacagtaccaccgaagtcggtgatgctgtcgccgaagaagttaagaaaatccttgcttaaaaagattctctttttttatgatatttgtacataaactttataaatgaaattcataatagaaacgacacgaaattacaaaatggaatatgttcatagggtaacgctatgatccaatatcaaaggaaatgatagcattgaaggatgagactaatccaattgaggagtggcagcatatagaacagctaaagggtagtgctgaaggaagcatacgataccccgcatggaatgggataatatcacaggaggtactagactacctttcatcctacataaatagacgcatataagtacgcatttaagcataaacacgcactatgccgttcttctcatgtatatatatatacaggcaacacgcagatataggtgcgacgtgaacagtgagctgtatgtgcgcagctcgcgttgcattttcggaagcgctcgttttcggaaacgctttgaagttcctattccgaagttcctattctctagaaagtataggaacttcagagcgcttttgaaaaccaaaagcgctctgaagtcgcactttcaaaaaaccaaaaacgcaccggactgtaacgagctactaaaatattgcgaataccgcttccacaaacattgctcaaaagtatctctttgctatatatctctgtgctatatccctatataacctacccatccacctttcgctccttgaacttgcatctaaactcgacctctacattttttatgtttatctctagtattactctttagacaaaaaaattgtagtaagaactattcatagagtgaatcgaaaacaatacgaaaatgtaaacatttcctatacgtagtatatagagacaaaatagaagaaaccgttcataattttctgaccaatgaagaatcatcaacgctatcactttctgttcacaaagtatgcgcaatccacatcggtatagaatataatcggggatgcctttatcttgaaaaaatgcacccgcagcttcgctagtaatcagtaaacgcgggaagtggagtcaggctttttttatggaagagaaaatagacaccaaagtagccttcttctaaccttaacggacctacagtgcaaaaagttatcaagagactgcattatagagcgcacaaaggagaaaaaaagtaatctaagatgctttgttagaaaaatagcgctctcgggatgcatttttgtagaacaaaaaagaagtatagattctttgttggtaaaatagcgctctcgcgttgcatttctgttctgtaaaaatgcagctcagattctttgtttgaaaaattagcgctctcgcgttgcatttttgttttacaaaaatgaagcacagattcttcgttggtaaaatagcgctttcgcgttgcatttctgttctgtaaaaatgcagctcagattctttgtttgaaaaattagcgctctcgcgttgcatttttgttctacaaaatgaagcacagatgcttcgttcaggtggcacttttcggggaaatgtgcgcggaacccctatttgtttatttttctaaatacattcaaatatgtatccgctcatgagacaataaccctgatattgg

SEQ ID NO: 35 - DNA, 6009 bp, Artificial Sequence
  pJ1234-03C plasmid
tcagaattggttaattggttgtaacactgacccctatttgtttatttttctaaatacattcaaatatgtatccgctcatgagacaataaccctgataaatgcttcaataatattgaaaaaggaagaatatgagtattcaacatttccgtgtcgcccttattcccttttttgcggcattttgccttcctgtttttgctcacccagaaacgctggtgaaagtaaaagatgctgaagatcagttgggtgcacgagtgggttacatcgaactggatctcaacagcggtaagatccttgagagttttcgccccgaagaacgttttccaatgatgagcacttttaaagttctgctatgtggcgcggtattatcccgtattgacgccgggcaagagcaactcggtcgccgcatacactattctcagaatgacttggttgagtactcaccagtcacagaaaagcatcttacggatggcatgacagtaagagaattatgcagtgctgccataaccatgagtgataacactgcggccaacttacttctgacaacgatcggaggaccgaaggagctaaccgcttttttgcacaacatgggggatcatgtaactcgccttgatcgttgggaaccggagctgaatgaagccataccaaacgacgagcgtgacaccacgatgcctgtagcgatggcaacaacgttgcgcaaactattaactggcgaactacttactctagcttcccggcaacaattaatagactggatggaggcggataaagttgcaggaccacttctgcgctcggcccttccggctggctggtttattgctgataaatccggagccggtgagcgtggttctcgcggtatcatcgcagcgctggggccagatggtaagccctcccgtatcgtagttatctacacgacggggagtcaggcaactatggatgaacgaaatagacagatcgctgagataggtgcctcactgattaagcattggtaactcatgaccaaaatcccttaacgtgagttacgcgcgcgtcgttccactgagcgtcagaccccgtagaaaagatcaaaggatcttcttgagatcctttttttctgcgcgtaatctgctgcttgcaaacaaaaaaaccaccgctaccagcggtggtttgtttgccggatcaagagctaccaactctttttccgaaggtaactggcttcagcagagcgcagataccaaatactgttcttctagtgtagccgtagttagcccaccacttcaagaactctgtagcaccgcctacatacctcgctctgctaatcctgttaccagtggctgctgccagtggcgataagtcgtgtcttaccgggttggactcaagacgatagttaccggataaggcgcagcggtcgggctgaacggggggttcgtgcacacagcccagcttggagcgaacgacctacaccgaactgagatacctacagcgtgagctatgagaaagcgccacgcttcccgaagggagaaaggcggacaggtatccggtaagcggcagggtcggaacaggagagcgcacgagggagcttccagggggaaacgcctggtatctttatagtcctgtcgggtttcgccacctctgacttgagcgtcgatttttgtgatgctcgtcaggggggcggagcctatggaaaaacgccagcaacgcggcctttttacggttcctggccttttgctggccttttgctcacatgttctttcctgcgttatcccctgattctgtggataaccgtattaccgcctttgagtgagctgataccgctcggggtcgtgcaggtagtttatcattatcaatactcgccatttcaaagaatacgtaaataattaatagtagtgattttcctaactttatttagtcaaaaaattagccttttaattctgctgtaacccgtacatgcccaaaatagggggcgggttacacagaatatataacatcgtaggtgtctgggtgaacagtttattcctggcatccactaaatataatggagcccgctttttaagctggcatccagaaaaaaaaagaatcccagcaccaaaatattgttttcttcaccaaccatcagttcataggtccattctcttagcgcaactacagagaacaggggcacaaacaggcaaaaaacgggcacaacctcaatggagtgatgcaaccagcctggagtaaatgatgacacaaggcaattgacccacgcatgtatctatctcattttcttacaccttctattaccttctgctctctctgatttggaaaaagctgaaaaaaaaggttgaaaccagttccctgaaattattcccctacttgactaataagtatataaagacggtaggtattgattgtaattctgtaaatctatttcttaaacttcttaaattctacttttatagttagtcttttttttagttttaaaacaccagaacttagtttcgacggataaaatgacagctttaactgaaggggccaagcttttcgaaaaagagatcccatatatcaccgaacttgaaggtgacgttgagggtatgaagtttatcataaaaggagaaggcacaggtgatgcgacaacgggtacaatcaaggcaaagtacatttgtacaactggggacctgcctgtcccatgggccactttggtgtctactttgtcttacggcgtacaatgttttgctaagtacccttcacacatcaaagatttctttaagtctgcaatgcctgaaggatacacacaggaacgtacaatttcatttgagggcgacggtgtctataaaacaagagctatggttacttatgaaagaggttccatctacaacagagtgacactaacgggcgaaaatttcaaaaaggatggacatattttgcgtaaaaacgtagctttccaatgcccaccatcaatactatacattctgccagatactgtaaacaatggtattagagtcgagtttaatcaagcttatgatatagaaggtgtcactgaaaaattggttacaaaatgcagccaaatgaatagaccattggcaggatctgccgctgtgcatatccctagataccatcacattacctaccacaccaaattaagtaaagacagggatgaacgaagagatcatatgtgtttagttgaggttgttaaggcagttgatctcgacacttaccaataaatcatgtaattagttatgtcacgcttacattcacgccctccccccacatccgctctaaccgaaaaggaaggagttagacaacctgaagtctaggtccctatttatttttttatagttatgttagtattaagaacgttatttatatttcaaatttttcttttttttctgtacagacgcgtgtacgcatgtaacattatactgaaaaccttgcttgagaaggttttgggacgctcgaaggctttaatttgcggcccctcacctgcacgcaaaaagcttttcaattcaattcatcattttttttttattcttttttttgatttcggtttctttgaaatttttttgattcggtaatctccgaacagaaggaagaacgaaggaaggagcacagacttagattggtatatatacgcatatgtagtgttgaagaaacatgaaattgcccagtattcttaacccaactgcacagaacaaaaaccagcaggaaacgaagataaatcatgtcgaaagctacatataaggaacgtgctgctactcatcctagtcctgttgctgccaagctatttaatatcatgcacgaaaagcaaacaaacttgtgtgcttcattggatgttcgtaccaccaaggaattactggagttagttgaagcattaggtcccaaaatttgtttactaaaaacacatgtggatatcttgactgatttttccatggagggcacagttaagccgctaaaggcattatccgccaagtacaattttttactcttcgaagatagaaaatttgctgacattggtaatacagtcaaattgcagtactctgcgggtgtatacagaatagcagaatgggcagacattacgaatgcacacggtgtggtgggcccaggtattgttagcggtttgaagcaggcggcagaagaagtaacaaaggaacctagaggccttttgatgttagcagaattgtcatgcaagggctccctatctactggagaatatactaagggtactgttgacattgcgaaaagcgacaaagattttgttatcggctttattgctcaaagagacatgggtggaagagatgaaggttacgattggttgattatgacacccggtgtgggtttagatgacaagggagatgcattgggtcaacagtatagaaccgtggatgatgttgtctctacaggatctgacattattattgttggaagaggactatttgcaaagggaagggatgctaaggtagagggtgaacgttacagaaaagcaggctgggaagcatatttgagaagatgcggccagcaaaactaaaaaactgtattataagtaaatgcatgtatactaaactcacaaattagagcttcaatttaattatatcagttattacccacgctatgatccaatatcaaaggaaatgatagcattgaaggatgagactaatccaattgaggagtggcagcatatagaacagctaaagggtagtgctgaaggaagcatacgataccccgcatggaatgggataatatcacaggaggtactagactacctttcatcctacataaatagacgcatataagtacgcatttaagcataaacacgcactatgccgttcttctcatgtatatatatatacaggcaacacgcagatataggtgcgacgtgaacagtgagctgtatgtgcgcagctcgcgttgcattttcggaagcgctcgttttcggaaacgctttgaagttcctattccgaagttcctattctctagaaagtataggaacttcagagcgcttttgaaaaccaaaagcgctctgaagtcgcactttcaaaaaaccaaaaacgcaccggactgtaacgagctactaaaatattgcgaataccgcttccacaaacattgctcaaaagtatctctttgctatatatctctgtgctatatccctatataacctacccatccacctttcgctccttgaacttgcatctaaactcgacctctacattttttatgtttatctctagtattactctttagacaaaaaaattgtagtaagaactattcatagagtgaatcgaaaacaatacgaaaatgtaaacatttcctatacgtagtatatagagacaaaatagaagaaaccgttcataattttctgaccaatgaagaatcatcaacgctatcactttctgttcacaaagtatgcgcaatccacatcggtatagaatataatcggggatgcctttatcttgaaaaaatgcacccgcagcttcgctagtaatcagtaaacgcgggaagtggagtcaggctttttttatggaagagaaaatagacaccaaagtagccttcttctaaccttaacggacctacagtgcaaaaagttatcaagagactgcattatagagcgcacaaaggagaaaaaaagtaatctaagatgctttgttagaaaaatagcgctctcgggatgcatttttgtagaacaaaaaagaagtatagattctttgttggtaaaatagcgctctcgcgttgcatttctgttctgtaaaaatgcagctcagattctttgtttgaaaaattagcgctctcgcgttgcatttttgttttacaaaaatgaagcacagattcttcgttggtaaaatagcgctttcgcgttgcatttctgttctgtaaaaatgcagctcagattctttgtttgaaaaattagcgctctcgcgttgcatttttgttctacaaaatgaagcacagatgcttcgttcaggtggcacttttcggggaaatgtgcgcggaacccctatttgtttatttttctaaatacattcaaatatgtatccgctcatgagacaataaccctgatattgg

SEQ ID NO: 36 - DNA, 42 bp, Artificial Sequence
  BsaI-AraC-MnP-H4_FT primer
taacttggtctcagggggccgtcaattgtctgattcgttacc

SEQ ID NO: 37 - DNA, 63 bp, Artificial Sequence
  MnP-H4_FT-6xHis-reverse primer
tgatgcctggctctagtattagtgatggtgatggtgatgcgccggaccgtcgaattgcacacc

SEQ ID NO: 38 - DNA, 38 bp, Artificial Sequence
  MnP-H4_FT-6xHis-forward primer
catcaccatcaccatcactaatactagagccaggcatc

SEQ ID NO: 39 - DNA, 66 bp, Artificial Sequence
  ChuA-6xHis-BsaI primer
tctaacttttagagaccttagtggtgatggtggtggtgccattggtaggaaacgaaaatcttgccg

SEQ ID NO: 40 - DNA, 4569 bp, Artificial Sequence
  AraC-MnP-H4_FT-ChuA PCR product
gggggccgtcaattgtctgattcgttaccaattatgacaacttgacggctacatcattcactttttcttcacaaccggcacggaactcgctcgggctggccccggtgcattttttaaatacccgcgagaaatagagttgatcgtcaaaaccaacattgcgaccgacggtggcgataggcatccgggtggtgctcaaaagcagcttcgcctggctgatacgttggtcctcgcgccagcttaagacgctaatccctaactgctggcggaaaagatgtgacagacgcgacggcgacaagcaaacatgctgtgcgacgctggcgatatcaaaattgctgtctgccaggtgatcgctgatgtactgacaagcctcgcgtacccgattatccatcggtggatggagcgactcgttaatcgcttccatgcgccgcagtaacaattgctcaagcagatttatcgccagcagctccgaatagcgcccttccccttgcccggcgttaatgatttgcccaaacaggtcgctgaaatgcggctggtgcgcttcatccgggcgaaagaaccccgtattggcaaatattgacggccagttaagccattcatgccagtaggcgcgcggacgaaagtaaacccactggtgataccattcgcgagcctccggatgacgaccgtagtgatgaatctctcctggcgggaacagcaaaatatcacccggtcggcaaacaaattctcgtccctgatttttcaccaccccctgaccgcgaatggtgagattgagaatataacctttcattcccagcggtcggtcgataaaaaaatcgagataaccgttggcctcaatcggcgttaaacccgccaccagatgggcattaaacgagtatcccggcagcaggggatcattttgcgcttcagccatacttttcatactcccgccattcagagaagaaaccaattgtccatattgcatcagacattgccgtcactgcgtcttttactggctcttctcgctaaccaaaccggtaaccccgcttattaaaagcattctgtaacaaagcgggaccaaagccatgacaaaaacgcgtaacaaaagtgtctataatcacggcagaaaagtccacattgattatttgcacggcgtcacactttgctatgccatagcatttttatccataagattagcggatcctacctgacgctttttatcgcaactctctactgtttctccatacccgtttttttgggctagcaggaggaattcaccatggcagtatgtccagacggtaccagagtgacgaatgcagcgtgttgcgcgttcattccgctggcgcaggatctgcaggaaaccctgttccaaggcgattgcggcgaggacgcgcacgaggtcattcgcctgacctttcacgatgccattgcaatcagccagtctttgggtccgcaagcgggtggtggcgcggacggcagcatgttgcactttccgaccatcgagccgaatttctcggccaatagcggtattgacgatagcgttaacaacctgttgccgtttatgcaaaagcatgacaccatcagcgctgcggacctggttcagttcgcaggcgccgtggcgctgagcaactgtcctggtgcgccacgtctggagttcatggcgggtcgcccgaataccacgatcccggcagttgaaggtctgattccggagccgcaggacagcgtcaccaaaattctgcagcgtttcgaggatgccggtaactttagcccgttcgaggtcgtgagcctgttggcgagccatacggtggcgcgtgctgacaaagttgatgaaaccatcgacgccgctccgttcgacagcaccccgtttacgtttgatacccaggttttcctggaagttctgttgaaaggcaccggctttccgggttccaataacaacaccggtgaagtcatgtctccgctgcctctgggctcgggtagcgatactggtgagatgcgcctgcaaagcgactttgctctggcccgtgatgagcgtaccgcgtgcttctggcagtccttcgtcaacgaacaagagtttatggcggccagctttaaggctgcgatggcaaaactggcaattctgggccatagccgttccagcctgatcgattgcagcgacgtggttccggtgccgaagcctgcggtcaataagccggcgaccttcccggcgaccaaaggcccgaaggacctggatactctgacgtgtaaagcgctgaagtttccgacgctgacgtctgatccgggtgccacggagactctgatcccgcactgcagcaatggtggcatgagctgcccgggtgtgcaattcgacggtccggcgcatcaccatcaccatcactaatactagagccaggcatcaaataaaacgaaaggctcagtcgaaagactgggcctttcgttttatctgttgtttgtcggtgaacgctctctactagagtcacactggctcaccttcgggtgggcctttctgcgtttatagtcgacttgacagctagctcagtcctaggtattgtgctagctactagagaaagaggagaaatactagatgtcccgccctcaattcacctcgctccgtttgtctttgctcgcactcgccgtatccgcaacgctgccgacctttgccttcgctaccgaaaccatgaccgttaccgcgaccggcaacgcacgcagctcgttcgaggcgccgatgatggtgagcgtgatcgatacctctgctccggagaaccagacggcgacgagcgctaccgatctgctgcgccacgtgccgggtattacgctggacggtaccggtcgcacgaacggtcaagacgtgaacatgcgcggctacgaccatcgcggtgtgctggtcctggtcgatggtgtgcgtcagggtacggataccggtcacttgaatggtacctttctggatccggcgctgattaagcgtgtcgaaatcgtgcgtggcccgtcggcactgctgtatggtagcggtgcgctgggcggtgtgatcagctacgataccgtcgatgcgaaagacctgttgcaagagggtcaaagctccggtttccgcgtttttggtactggtggtaccggtgaccatagcctgggcctgggcgcgagcgcgtttggtcgcacggaaaacctggatggcatcgttgcgtggagcagccgtgatcgtggtgacttgcgccagtctaatggcgaaacggcccctaacgatgaaagcattaacaacatgctggccaagggtacgtggcagatcgatagcgcgcagagcctgagcggcctggtccgttactacaacaacgacgcgcgtgagccgaaaaacccgcagacggtcgaggcgagcgagagcagcaacccgatggtggaccgtagcaccattcaacgtgatgcccaactgagctataagctggcaccgcaaggtaatgactggctgaatgcggatgcgaaaatctactggagcgaagttcgcatcaatgcacagaatacgggtagctctggcgagtaccgtgaacagattaccaaaggtgcacgtctggagaatcgttctacgctgtttgctgacagcttcgcttcgcatctgctgacgtatggtggcgagtattatcgtcaggaacaacacccaggtggtgcgaccacgggtttcccgcaggcgaagatcgattttagcagcggctggctgcaagatgagatcaccttgcgtgacttgccgattaccctgctgggtggtacgcgttatgacagctaccgtggcagcagcgacggttacaaagacgtcgatgcagataaatggagctcccgtgccggcatgaccattaatccgaccaattggctgatgctgttcggcagctatgcgcaagcgttccgtgccccaaccatgggtgagatgtacaatgacagcaagcatttcagcattggtcgcttctacacgaattactgggtgccgaacccgaatctgcgtccggagactaatgaaacccaggagtatggttttggcctgcgctttgatgatctgatgctgagcaacgacgccctggaattcaaggcgagctactttgacactaaagccaaagactacattagcactacggttgattttgcggctgctaccaccatgtcctataatgttccaaacgcaaagatttggggctgggacgtcatgaccaagtacaccaccgacctgtttagcttggatgttgcatacaatcgcacccgtggcaaagacaccgataccggcgaatacatcagcagcatcaatccggacaccgttacgtccaccctgaacatcccgattgcgcacagcggtttcagcgttggttgggttggtacgtttgcggatcgctccacccacatctcgtcgtcttatagcaagcaaccgggctacggcgtgaatgatttctatgtgagctatcagggccagcaagccctgaaaggtatgacgactaccctggttctgggcaacgcattcgacaaagagtattggagcccgcagggcattccgcaggacggtcgtaacggcaagattttcgtttcctaccaatggcaccaccaccatcaccactaaggtctctaaaa

SEQ ID NO: 41 - DNA, 42 bp, Artificial Sequence
  BsaI-PrpR-PDI primer
taacttggtctcaggggtcagcttttcagccgccgccagaac

SEQ ID NO: 42 - DNA, 55 bp, Artificial Sequence
  PDI-5xHis-BsaI primer
tctaacttttagagaccttagtggtggtggtggtgcagctcatcgtgctccgtcg

SEQ ID NO: 43 - DNA, 3326 bp, Artificial Sequence
  PrpR-PDI PCR product
ggggtcagcttttcagccgccgccagaacgtcgtccggctgatgcctaaataattcgccgctgctgttttatcgccattaaatttctccagtgcctgttgtggtgtcagtaagcgtggagcgggagttttcgccgactcgcgcgccagttccggcagtagcagttgcataaactgcggcgttaaatccggcgtcggttccacacttaaaaacagcgccagtcgttccatcatattgcgcagttcacgaatattgcctggccagtcgtagtgcagcagcacagtttcacttgcctgtaacccctggcgtaatgcagcagaaaatggggcggagagcgccgccagagacactttcaaaaagctttccgccagcggaagaatatccgccacccgctcgcgcagtggtggcaattgcagacgcaaaatactcagccgataaaacagatcacggcgaaaacgtccttgctgcatatcttcttccagattgcagtgagtggcgctaatgacccgtacatctaccggaacaggctgatgcccgccgacgcgggtgacctctttttcttccagcacccgcagcagccgggtctgcaaaggtagcggcatttcgccaatctcatccagaaacagcgtaccgccgtgggcaatttcgaacagcccggcgcgacctccgcgtcgcgagccggtaaacgccccttcctcatagccaaacagttctgcttccagcagcgattcggcaatcgccccgcagttgacggcaacaaacggatgcgactttttgccctgtcgcgcatcgtggcgggcaaaatattcccgatgaatcgcctgggccgccagctctttgcccgtccccgtttccccctcaatcaacaccgccgcactggagcgggcatacagcaaaatagtctgccgtacttgttccatctgtggtgattgaccgagcatatcgcccagcacgtaacgagtacgcagggcgttgcgggtggcatcgtgagtgttatggcgtaacgacatgcgcgtcatatccagcgcatcgctgaacgcctggcgcacggtggcggcggaatagataaaaattccggtcattccggcttcttctgccaaatcggtaatcagccctgcgccgaccaccgcttcggtgccgttagcttttagctcgttaatctgcccgcgtgcgtcttcctcggtaatgtagctacgttggtcgaggcgcaaattaaaggttttttgaaacgccaccagcgctggaatggtttcctgataggtgacaacgccgatagaagaggtgagttttccggcttttgccagtgcctgtaacacatcgtagccgctcggtttaatcaaaataactggcactgacaggcggcttttcaggtacgcgccgttagagccagccgcgatgatggcgtcacagcgttcgtttgccagtttcttgcggatgtaggtcactgctttttcaaagccaagctgaataggggtaatgttcgccaggtgatcaaactcgaggctgatatcgcgaaacagctcgaacaggcgcgttacagataccgtccagataaccggtttgtcgtcattaagccgtggtggatgtgccatagcgcaccgcaaagttaagaaaccgaatattgggtttagtcttgtttcataattgttgcaatgaaacgcggtgaaacattgcctgaaacgttaactgaaacgcatatttgcggattagttcatgactttatctctaacaaattgaaattaaacatttaattttattaaggcaattgtggcacaccccttgctttgtctttatcaacgcaaataacaagttgataacaagctagcaggaggaattcaccatgtctgatgttgtacaactgaagaaagatacgttcgatgactttatcaaaactaatgacttggtgctggcagagtttttcgccccgtggtgtggccactgcaaagctctggctccggagtacgaagaggccgcgaccaccctgaaagaaaagaacatcaaactggcgaaagtggactgtacggaagaaaccgacctgtgtcagcagcacggcgtggaaggttacccgaccctgaaggtgtttcgtggcctggacaatgttagcccgtacaaaggtcaacgtaaggccgcagcgatcaccagctacatgatcaagcagtcgctgcctgcagtctctgaggtgaccaaagataatctggaagagttcaaaaaggcagataaggcggtgctggttgcctatgttgatgcaagcgacaaggcgagcagcgaggtctttacccaggtcgcggagaaattgcgcgataactacccgttcggcagcagctccgatgcagctttggccgaggcggaaggtgtcaaggctccggcgatcgttctgtacaaagatttcgacgagggtaaagcggtgttcagcgaaaagtttgaggtggaagcaattgaaaagttcgcaaaaaccggtgccacgcctttgattggcgaaatcggtccggaaacctattctgactatatgagcgccggtatcccgctggcctacattttcgcagaaacggcagaagagcgcaaagaactgagcgacaagttgaagccaattgcagaggcacagcgtggcgtcatcaactttggtaccattgacgcgaaagcatttggtgcgcatgccggtaacctgaatctgaaaacggacaaatttccggcgtttgcgattcaagaggtggcgaagaaccaaaagtttccgttcgatcaagaaaaagagattaccttcgaggcgatcaaagcgttcgttgacgactttgttgccggtaaaatcgagccgagcattaagagcgagccgatcccggagaagcaggaaggcccggtgaccgtcgtcgtcgcgaagaattacaacgagattgttctggatgacacgaaagacgtcctgattgagttctatgcgccgtggtgcggtcattgcaaagcgctggccccgaaatatgaagagctgggtgcgctgtacgcgaagagcgagtttaaggaccgtgtggttatcgcgaaagtagatgcgaccgccaatgacgttcctgacgagatccaaggcttcccgaccattaaactgtatccggctggtgctaaaggccagccagttacctatagcggtagccgcacggttgaggatctgattaagttcattgccgagaacggcaagtacaaggcggcaatcagcgaggatgcagaagaaacgagctccgcaaccgaaaccacgacggaaaccgctactaagtccgaagaggcggcgaaagaaaccgcgacggagcacgatgagctgcaccaccaccaccactaaggtctctaaaa

SEQ ID NO: 44 - DNA, 44 bp, Artificial Sequence
  BsaI-AraC-HC-forward primer
taacttggtctcaggggaagccgtcaattgtctgattcgttacc

SEQ ID NO: 45 - DNA, 46 bp, Artificial Sequence
  HC-reverse primer
gctttgttgcagttgaacttccatggtgaattcctcctgctagccc

SEQ ID NO: 46 - DNA, 46 bp, Artificial Sequence
  HC-forward primer
gggctagcaggaggaattcaccatggaagttcaactgcaacaaagc

SEQ ID NO: 47 - DNA, 45 bp, Artificial Sequence
  HC-BsaI-reverse primer
tctaacttttagagaccaagcttttatttacccggcgagtgggac

SEQ ID NO: 48 - DNA, 43 bp, Artificial Sequence
  BsaI-PrpR-LC-forward primer
taacttggtctcagggggcgtagaggatctgctcatgtttgac

SEQ ID NO: 49 - DNA, 50 bp, Artificial Sequence
  LC-reverse primer
cgcttgcgtcataacaatatcagccatggtgaattcctcctgctagcttg

SEQ ID NO: 50 - DNA, 50 bp, Artificial Sequence
  LC-forward primer
caagctagcaggaggaattcaccatggctgatattgttatgacgcaagcg

SEQ ID NO: 51 - DNA, 43 bp, Artificial Sequence
  LC-BsaI-reverse primer
tctaacttttagagacctctctcatccgccaaaacagccaagc

SEQ ID NO: 52 - DNA, 2615 bp, Artificial Sequence
  AraC-HC_NS PCR product
ggggaagccgtcaattgtctgattcgttaccaattatgacaacttgacggctacatcattcactttttcttcacaaccggcacggaactcgctcgggctggccccggtgcattttttaaatacccgcgagaaatagagttgatcgtcaaaaccaacattgcgaccgacggtggcgataggcatccgggtggtgctcaaaagcagcttcgcctggctgatacgttggtcctcgcgccagcttaagacgctaatccctaactgctggcggaaaagatgtgacagacgcgacggcgacaagcaaacatgctgtgcgacgctggcgatatcaaaattgctgtctgccaggtgatcgctgatgtactgacaagcctcgcgtacccgattatccatcggtggatggagcgactcgttaatcgcttccatgcgccgcagtaacaattgctcaagcagatttatcgccagcagctccgaatagcgcccttccccttgcccggcgttaatgatttgcccaaacaggtcgctgaaatgcggctggtgcgcttcatccgggcgaaagaaccccgtattggcaaatattgacggccagttaagccattcatgccagtaggcgcgcggacgaaagtaaacccactggtgataccattcgcgagcctccggatgacgaccgtagtgatgaatctctcctggcgggaacagcaaaatatcacccggtcggcaaacaaattctcgtccctgatttttcaccaccccctgaccgcgaatggtgagattgagaatataacctttcattcccagcggtcggtcgataaaaaaatcgagataaccgttggcctcaatcggcgttaaacccgccaccagatgggcattaaacgagtatcccggcagcaggggatcattttgcgcttcagccatacttttcatactcccgccattcagagaagaaaccaattgtccatattgcatcagacattgccgtcactgcgtcttttactggctcttctcgctaaccaaaccggtaaccccgcttattaaaagcattctgtaacaaagcgggaccaaagccatgacaaaaacgcgtaacaaaagtgtctataatcacggcagaaaagtccacattgattatttgcacggcgtcacactttgctatgccatagcatttttatccataagattagcggatcctacctgacgctttttatcgcaactctctactgtttctccatacccgtttttttgggctagcaggaggaattcaccatggaagttcaactgcaacaaagcggtccggaactgattaaaccgggcgcgagcgtgaagatgtcttgcaaagccagtggttacacctttacgtcttatgtgatgcattgggttaaacagaagccgggccaaggtctggaatggattggctacatcaacccgtacaacgatggtaccaagtacaacgaaaagttcaagggcaaagcaaccctgacgagtgacaaaagctctagtacggcttatatggaactgtcctcactgacctcagaagattcggcagtgtattactgcgctcgtggcacgtattactatggttcccgcgtttttgattactggggccagggtaccacgctgaccgtttcgagcgcgaaaaccacgccgccgagcgtctatccgctggcaccgggttcggcagcacagacgaatagcatggtgaccctgggctgtctggttaaaggttactttccggaaccggtgaccgttacgtggaacagcggctctctgtctagtggtgtccatacgttcccggcggtgctgcagtctgatctgtataccctgtcctcatcggtcacggtgccgagctctacctggccgagtgaaaccgtcacgtgcaacgtggcacacccggcaagttccaccaaagttgataaaaagattgtcccgcgtgactgcggctgtaaaccgtgcatctgtaccgtgccggaagtttcatcggtctttattttcccgccgaagccgaaagatgtcctgaccatcacgctgaccccgaaggtgacctgtgtggttgtcgacatttctaaagatgacccggaagttcagtttagttggttcgtcgatgacgttgaagtccatacggcgcagacccaaccgcgtgaagaacagtttaatagcaccttccgcagtgtgtccgaactgccgatcatgcaccaagactggctgaatggcaaggaatttaaatgccgtgttaactcggcagctttcccggccccgattgaaaagacgatcagcaagaccaaaggtcgcccgaaagcaccgcaggtgtataccattccgccgccgaaagaacaaatggctaaggataaagttagcctgacgtgtatgattaccgatttctttccggaagacatcaccgtggaatggcagtggaacggccaaccggccgaaaactataaaaatacgcagccgatcatggataccgacggttcctactttgtgtattcaaagctgaacgttcaaaaatccaattgggaagccggtaacacgttcacctgttcagttctgcacgaaggtctgcacaatcaccatacggaaaagtcgctgtcccactcgccgggtaaataaaagcttggtctctaaaa

SEQ ID NO: 53 - DNA, 2584 bp, Artificial Sequence
  PrpR-LC_NS PCR product
gggggcgtagaggatctgctcatgtttgacagcttatcatcgattcagcttttcagccgccgccagaacgtcgtccggctgatgcctaaataattcgccgctgctgttttatcgccattaaatttctccagtgcctgttgtggtgtcagtaagcgtggagcgggagttttcgccgactcgcgcgccagttccggcagtagcagttgcataaactgcggcgttaaatccggcgtcggttccacacttaaaaacagcgccagtcgttccatcatattgcgcagttcacgaatattgcctggccagtcgtagtgcagcagcacagtttcacttgcctgtaacccctggcgtaatgcagcagaaaatggggcggagagcgccgccagagacactttcaaaaagctttccgccagcggaagaatatccgccacccgctcgcgcagtggtggcaattgcagacgcaaaatactcagccgataaaacagatcacggcgaaaacgtccttgctgcatatcttcttccagattgcagtgagtggcgctaatgacccgtacatctaccggaacaggctgatgcccgccgacgcgggtgacctctttttcttccagcacccgcagcagccgggtctgcaaaggtagcggcatttcgccaatctcatccagaaacagcgtaccgccgtgggcaatttcgaacagcccggcgcgacctccgcgtcgcgagccggtaaacgccccttcctcatagccaaacagttctgcttccagcagcgattcggcaatcgccccgcagttgacggcaacaaacggatgcgactttttgccctgtcgcgcatcgtggcgggcaaaatattcccgatgaatcgcctgggccgccagctctttgcccgtccccgtttccccctcaatcaacaccgccgcactggagcgggcatacagcaaaatagtctgccgtacttgttccatctgtggtgattgaccgagcatatcgcccagcacgtaacgagtacgcagggcgttgcgggtggcatcgtgagtgttatggcgtaacgacatgcgcgtcatatccagcgcatcgctgaacgcctggcgcacggtggcggcggaatagataaaaattccggtcattccggcttcttctgccaaatcggtaatcagccctgcgccgaccaccgcttcggtgccgttagcttttagctcgttaatctgcccgcgtgcgtcttcctcggtaatgtagctacgttggtcgaggcgcaaattaaaggttttttgaaacgccaccagcgctggaatggtttcctgataggtgacaacgccgatagaagaggtgagttttccggcttttgccagtgcctgtaacacatcgtagccgctcggtttaatcaaaataactggcactgacaggcggcttttcaggtacgcgccgttagagccagccgcgatgatggcgtcacagcgttcgtttgccagtttcttgcggatgtaggtcactgctttttcaaagccaagctgaataggggtaatgttcgccaggtgatcaaactcgaggctgatatcgcgaaacagctcgaacaggcgcgttacagataccgtccagataaccggtttgtcgtcattaagccgtggtggatgtgccatagcgcaccgcaaagttaagaaaccgaatattgggtttagtcttgtttcataattgttgcaatgaaacgcggtgaaacattgcctgaaacgttaactgaaacgcatatttgcggattagttcatgactttatctctaacaaattgaaattaaacatttaattttattaaggcaattgtggcacaccccttgctttgtctttatcaacgcaaataacaagttgataacaagctagcaggaggaattcaccatggctgatattgttatgacgcaagcggctccgtctattccggttaccccgggtgaaagcgtctctatcagttgccgcagctctaaatcgctgctgaacagcaatggtaacacctatctgtactggtttctgcagcgtccgggtcagagcccgcaactgctgatttatcgcatgtctaatctggcaagtggtgtcccggatcgtttttccggttcaggttcgggtacggcattcaccctgcgtatctcccgcgttgaagccgaagacgtcggcgtgtattactgcatgcagcatctggaatacccgtttacgttcggtgcaggcaccaaactggaactgaaacgcgctgatgcagcaccgaccgtgagcattttcccgccgagttccgaacaactgacctccggcggtgcatcagtggtttgttttctgaacaacttctacccgaaagatatcaacgtgaaatggaaaatcgacggttcggaacgtcagaatggcgttctgaacagctggacggatcaagacagtaaagattccacctactcaatgtcatcgaccctgacgctgaccaaagacgaatatgaacgccataactcttacacgtgcgaagctacccacaaaacgagcacctctccgatcgttaaaagttttaatcgtaacgaatgttaaaagcttggctgttttggcggatgagagaggtctctaaaa